European Patent Application EP 4 495 597 A2, published January 22, 2025. Title: ANTI-TISSUE FACTOR ANTIBODIES, ANTIBODY-DRUG CONJUGATES, AND RELATED METHODS. Applicant: ICONIC THERAPEUTICS LLC. The sequence listing filed with the application follows.

SEQUENCE LISTING (922 sequences)

SEQ ID NO: 1 - protein, 10 aa, synthetic construct
  REGION 1..10: note = Description of Artificial Sequence: Synthetic peptide
GFTFSDYAMG

SEQ ID NO: 2 - protein, 17 aa, synthetic construct
  REGION 1..17: note = Description of Artificial Sequence: Synthetic peptide
TISGSGGLTYYADSVKG

SEQ ID NO: 3 - protein, 9 aa, synthetic construct
  REGION 1..9: note = Description of Artificial Sequence: Synthetic peptide
APYGYYMDV

SEQ ID NO: 4 - protein, 11 aa, synthetic construct
  REGION 1..11: note = Description of Artificial Sequence: Synthetic peptide
RASQSISSWLA

SEQ ID NO: 5 - protein, 7 aa, synthetic construct
  REGION 1..7: note = Description of Artificial Sequence: Synthetic peptide
KASSLES

SEQ ID NO: 6 - protein, 8 aa, synthetic construct
  REGION 1..8: note = Description of Artificial Sequence: Synthetic peptide
QQYKSYIT

SEQ ID NO: 7 - protein, 5 aa, synthetic construct
  REGION 1..5: note = Description of Artificial Sequence: Synthetic peptide
DYAMG

SEQ ID NO: 8 - protein, 17 aa, synthetic construct
  REGION 1..17: note = Description of Artificial Sequence: Synthetic peptide
TISGSGGLTYYADSVKG

SEQ ID NO: 9 - protein, 9 aa, synthetic construct
  REGION 1..9: note = Description of Artificial Sequence: Synthetic peptide
APYGYYMDV

SEQ ID NO: 10 - protein, 11 aa, synthetic construct
  REGION 1..11: note = Description of Artificial Sequence: Synthetic peptide
RASQSISSWLA

SEQ ID NO: 11 - protein, 7 aa, synthetic construct
  REGION 1..7: note = Description of Artificial Sequence: Synthetic peptide
KASSLES

SEQ ID NO: 12 - protein, 8 aa, synthetic construct
  REGION 1..8: note = Description of Artificial Sequence: Synthetic peptide
QQYKSYIT

SEQ ID NO: 13 - protein, 7 aa, synthetic construct
  REGION 1..7: note = Description of Artificial Sequence: Synthetic peptide
GFTFSDY

SEQ ID NO: 14 - protein, 4 aa, synthetic construct
  REGION 1..4: note = Description of Artificial Sequence: Synthetic peptide
GSGG

SEQ ID NO: 15 - protein, 7 aa, synthetic construct
  REGION 1..7: note = Description of Artificial Sequence: Synthetic peptide
PYGYYMD

SEQ ID NO: 16 - protein, 7 aa, synthetic construct
  REGION 1..7: note = Description of Artificial Sequence: Synthetic peptide
SQSISSW

SEQ ID NO: 17 - skipped

SEQ ID NO: 18 - protein, 5 aa, synthetic construct
  REGION 1..5: note = Description of Artificial Sequence: Synthetic peptide
YKSYI

SEQ ID NO: 19 - protein, 10 aa, synthetic construct
  REGION 1..10: note = Description of Artificial Sequence: Synthetic peptide
GFTFSDYAMG

SEQ ID NO: 20 - protein, 10 aa, synthetic construct
  REGION 1..10: note = Description of Artificial Sequence: Synthetic peptide
TISGSGGLTY

SEQ ID NO: 21 - protein, 9 aa, synthetic construct
  REGION 1..9: note = Description of Artificial Sequence: Synthetic peptide
APYGYYMDV

SEQ ID NO: 22 - protein, 11 aa, synthetic construct
  REGION 1..11: note = Description of Artificial Sequence: Synthetic peptide
RASQSISSWLA

SEQ ID NO: 23 - protein, 7 aa, synthetic construct
  REGION 1..7: note = Description of Artificial Sequence: Synthetic peptide
KASSLES

SEQ ID NO: 24 - protein, 8 aa, synthetic construct
  REGION 1..8: note = Description of Artificial Sequence: Synthetic peptide
QQYKSYIT

SEQ ID NO: 25 - protein, 6 aa, synthetic construct
  REGION 1..6: note = Description of Artificial Sequence: Synthetic peptide
SDYAMG

SEQ ID NO: 26 - protein, 13 aa, synthetic construct
  REGION 1..13: note = Description of Artificial Sequence: Synthetic peptide
WVSTISGSGGLTY

SEQ ID NO: 27 - protein, 10 aa, synthetic construct
  REGION 1..10: note = Description of Artificial Sequence: Synthetic peptide
AKAPYGYYMD

SEQ ID NO: 28 - protein, 7 aa, synthetic construct
  REGION 1..7: note = Description of Artificial Sequence: Synthetic peptide
SSWLAWY

SEQ ID NO: 29 - protein, 10 aa, synthetic construct
  REGION 1..10: note = Description of Artificial Sequence: Synthetic peptide
LLIYKASSLE

SEQ ID NO: 30 - protein, 7 aa, synthetic construct
  REGION 1..7: note = Description of Artificial Sequence: Synthetic peptide
QQYKSYI

SEQ ID NO: 31 - protein, 8 aa, synthetic construct
  REGION 1..8: note = Description of Artificial Sequence: Synthetic peptide
GFTFSDYA

SEQ ID NO: 32 - protein, 8 aa, synthetic construct
  REGION 1..8: note = Description of Artificial Sequence: Synthetic peptide
ISGSGGLT

SEQ ID NO: 33 - protein, 11 aa, synthetic construct
  REGION 1..11: note = Description of Artificial Sequence: Synthetic peptide
AKAPYGYYMDV

SEQ ID NO: 34 - protein, 6 aa, synthetic construct
  REGION 1..6: note = Description of Artificial Sequence: Synthetic peptide
QSISSW

SEQ ID NO: 35 - skipped

SEQ ID NO: 36 - protein, 8 aa, synthetic construct
  REGION 1..8: note = Description of Artificial Sequence: Synthetic peptide
QQYKSYIT

SEQ ID NO: 37 - protein, 118 aa, synthetic construct
  REGION 1..118: note = Description of Artificial Sequence: Synthetic polypeptide
EVQLLESGGGLVQPGGSLRLSCAASGFTFSDYAMGWVRQAPGKGLEWVSTISGSGGLTYYADSVKGRFTISRDNSKNTLYLQMNSLRAEDTAVYYCAKAPYGYYMDVWGKGTTVTVSS

SEQ ID NO: 38 - protein, 106 aa, synthetic construct
  REGION 1..106: note = Description of Artificial Sequence: Synthetic polypeptide
DIQMTQSPSTLSASVGDRVTITCRASQSISSWLAWYQQKPGKAPKLLIYKASSLESGVPSRFSGSGSGTEFTLTISSLQPDDFATYYCQQYKSYITFGGGTKVEIK

SEQ ID NO: 39 - protein, 10 aa, synthetic construct
  REGION 1..10: note = Description of Artificial Sequence: Synthetic peptide
GFTFSSYAMA

SEQ ID NO: 40 - protein, 17 aa, synthetic construct
  REGION 1..17: note = Description of Artificial Sequence: Synthetic peptide
AISGSGGLTYYADSVKG

SEQ ID NO: 41 - protein, 9 aa, synthetic construct
  REGION 1..9: note = Description of Artificial Sequence: Synthetic peptide
APYGYYMDV

SEQ ID NO: 42 - protein, 11 aa, synthetic construct
  REGION 1..11: note = Description of Artificial Sequence: Synthetic peptide
RASQSISSWLA

SEQ ID NO: 43 - protein, 7 aa, synthetic construct
  REGION 1..7: note = Description of Artificial Sequence: Synthetic peptide
KASSLES

SEQ ID NO: 44 - protein, 8 aa, synthetic construct
  REGION 1..8: note = Description of Artificial Sequence: Synthetic peptide
QQYKSYIT

SEQ ID NO: 45 - protein, 5 aa, synthetic construct
  REGION 1..5: note = Description of Artificial Sequence: Synthetic peptide
SYAMA

SEQ ID NO: 46 - protein, 17 aa, synthetic construct
  REGION 1..17: note = Description of Artificial Sequence: Synthetic peptide
AISGSGGLTYYADSVKG

SEQ ID NO: 47 - protein, 9 aa, synthetic construct
  REGION 1..9: note = Description of Artificial Sequence: Synthetic peptide
APYGYYMDV

SEQ ID NO: 48 - protein, 11 aa, synthetic construct
  REGION 1..11: note = Description of Artificial Sequence: Synthetic peptide
RASQSISSWLA

SEQ ID NO: 49 - protein, 7 aa, synthetic construct
  REGION 1..7: note = Description of Artificial Sequence: Synthetic peptide
KASSLES

SEQ ID NO: 50 - protein, 8 aa, synthetic construct
  REGION 1..8: note = Description of Artificial Sequence: Synthetic peptide
QQYKSYIT

SEQ ID NO: 51 - protein, 7 aa, synthetic construct
  REGION 1..7: note = Description of Artificial Sequence: Synthetic peptide
GFTFSSY

SEQ ID NO: 52 - protein, 4 aa, synthetic construct
  REGION 1..4: note = Description of Artificial Sequence: Synthetic peptide
GSGG

SEQ ID NO: 53 - protein, 7 aa, synthetic construct
  REGION 1..7: note = Description of Artificial Sequence: Synthetic peptide
PYGYYMD

SEQ ID NO: 54 - protein, 7 aa, synthetic construct
  REGION 1..7: note = Description of Artificial Sequence: Synthetic peptide
SQSISSW

SEQ ID NO: 55 - skipped

SEQ ID NO: 56 - protein, 5 aa, synthetic construct
  REGION 1..5: note = Description of Artificial Sequence: Synthetic peptide
YKSYI

SEQ ID NO: 57 - protein, 10 aa, synthetic construct
  REGION 1..10: note = Description of Artificial Sequence: Synthetic peptide
GFTFSSYAMA

SEQ ID NO: 58 - protein, 10 aa, synthetic construct
  REGION 1..10: note = Description of Artificial Sequence: Synthetic peptide
AISGSGGLTY

SEQ ID NO: 59 - protein, 9 aa, synthetic construct
  REGION 1..9: note = Description of Artificial Sequence: Synthetic peptide
APYGYYMDV

SEQ ID NO: 60 - protein, 11 aa, synthetic construct
  REGION 1..11: note = Description of Artificial Sequence: Synthetic peptide
RASQSISSWLA

SEQ ID NO: 61 - protein, 7 aa, synthetic construct
  REGION 1..7: note = Description of Artificial Sequence: Synthetic peptide
KASSLES

SEQ ID NO: 62 - protein, 8 aa, synthetic construct
  REGION 1..8: note = Description of Artificial Sequence: Synthetic peptide
QQYKSYIT

SEQ ID NO: 63 - protein, 6 aa, synthetic construct
  REGION 1..6: note = Description of Artificial Sequence: Synthetic peptide
SSYAMA

SEQ ID NO: 64 - protein, 13 aa, synthetic construct
  REGION 1..13: note = Description of Artificial Sequence: Synthetic peptide
WVSAISGSGGLTY

SEQ ID NO: 65 - protein, 10 aa, synthetic construct
  REGION 1..10: note = Description of Artificial Sequence: Synthetic peptide
AKAPYGYYMD

SEQ ID NO: 66 - protein, 7 aa, synthetic construct
  REGION 1..7: note = Description of Artificial Sequence: Synthetic peptide
SSWLAWY

SEQ ID NO: 67 - protein, 10 aa, synthetic construct
  REGION 1..10: note = Description of Artificial Sequence: Synthetic peptide
LLIYKASSLE

SEQ ID NO: 68 - protein, 7 aa, synthetic construct
  REGION 1..7: note = Description of Artificial Sequence: Synthetic peptide
QQYKSYI

SEQ ID NO: 69 - protein, 8 aa, synthetic construct
  REGION 1..8: note = Description of Artificial Sequence: Synthetic peptide
GFTFSSYA

SEQ ID NO: 70 - protein, 8 aa, synthetic construct
  REGION 1..8: note = Description of Artificial Sequence: Synthetic peptide
ISGSGGLT

SEQ ID NO: 71 - protein, 11 aa, synthetic construct
  REGION 1..11: note = Description of Artificial Sequence: Synthetic peptide
AKAPYGYYMDV

SEQ ID NO: 72 - protein, 6 aa, synthetic construct
  REGION 1..6: note = Description of Artificial Sequence: Synthetic peptide
QSISSW

SEQ ID NO: 73 - skipped

SEQ ID NO: 74 - protein, 8 aa, synthetic construct
  REGION 1..8: note = Description of Artificial Sequence: Synthetic peptide
QQYKSYIT

SEQ ID NO: 75 - protein, 118 aa, synthetic construct
  REGION 1..118: note = Description of Artificial Sequence: Synthetic polypeptide
EVQLLESGGGLVQPGGSLRLSCAASGFTFSSYAMAWVRQAPGKGLEWVSAISGSGGLTYYADSVKGRFTISRDNSKNTLYLQMNSLRAEDTAVYYCAKAPYGYYMDVWGKGTTVTVSS

SEQ ID NO: 76 - protein, 106 aa, synthetic construct; identical to SEQ ID NO: 38
  REGION 1..106: note = Description of Artificial Sequence: Synthetic polypeptide

SEQ ID NO: 77 - protein, 10 aa, synthetic construct
  REGION 1..10: note = Description of Artificial Sequence: Synthetic peptide
GYTFDVYGIS

SEQ ID NO: 78 - protein, 17 aa, synthetic construct
  REGION 1..17: note = Description of Artificial Sequence: Synthetic peptide
WIAPYNGNTNYAQKLQG

SEQ ID NO: 79 - protein, 14 aa, synthetic construct
  REGION 1..14: note = Description of Artificial Sequence: Synthetic peptide
DAGTYSPFGYGMDV

SEQ ID NO: 80 - protein, 11 aa, synthetic construct
  REGION 1..11: note = Description of Artificial Sequence: Synthetic peptide
RASQSISSWLA

SEQ ID NO: 81 - protein, 7 aa, synthetic construct
  REGION 1..7: note = Description of Artificial Sequence: Synthetic peptide
KASSLES

SEQ ID NO: 82 - protein, 10 aa, synthetic construct
  REGION 1..10: note = Description of Artificial Sequence: Synthetic peptide
QQFQSLPPFT

SEQ ID NO: 83 - protein, 5 aa, synthetic construct
  REGION 1..5: note = Description of Artificial Sequence: Synthetic peptide
VYGIS

SEQ ID NO: 84 - protein, 17 aa, synthetic construct
  REGION 1..17: note = Description of Artificial Sequence: Synthetic peptide
WIAPYNGNTNYAQKLQG

SEQ ID NO: 85 - protein, 14 aa, synthetic construct
  REGION 1..14: note = Description of Artificial Sequence: Synthetic peptide
DAGTYSPFGYGMDV

SEQ ID NO: 86 - protein, 11 aa, synthetic construct
  REGION 1..11: note = Description of Artificial Sequence: Synthetic peptide
RASQSISSWLA

SEQ ID NO: 87 - protein, 7 aa, synthetic construct
  REGION 1..7: note = Description of Artificial Sequence: Synthetic peptide
KASSLES

SEQ ID NO: 88 - protein, 10 aa, synthetic construct
  REGION 1..10: note = Description of Artificial Sequence: Synthetic peptide
QQFQSLPPFT

SEQ ID NO: 89 - protein, 7 aa, synthetic construct
  REGION 1..7: note = Description of Artificial Sequence: Synthetic peptide
GYTFDVY

SEQ ID NO: 90 - protein, 4 aa, synthetic construct
  REGION 1..4: note = Description of Artificial Sequence: Synthetic peptide
PYNG

SEQ ID NO: 91 - protein, 12 aa, synthetic construct
  REGION 1..12: note = Description of Artificial Sequence: Synthetic peptide
AGTYSPFGYGMD

SEQ ID NO: 92 - protein, 7 aa, synthetic construct
  REGION 1..7: note = Description of Artificial Sequence: Synthetic peptide
SQSISSW

SEQ ID NO: 93 - skipped

SEQ ID NO: 94 - protein, 7 aa, synthetic construct
  REGION 1..7: note = Description of Artificial Sequence: Synthetic peptide
FQSLPPF

SEQ ID NO: 95 - protein, 10 aa, synthetic construct
  REGION 1..10: note = Description of Artificial Sequence: Synthetic peptide
GYTFDVYGIS

SEQ ID NO: 96 - protein, 10 aa, synthetic construct
  REGION 1..10: note = Description of Artificial Sequence: Synthetic peptide
WIAPYNGNTN

SEQ ID NO: 97 - protein, 14 aa, synthetic construct
  REGION 1..14: note = Description of Artificial Sequence: Synthetic peptide
DAGTYSPFGYGMDV

SEQ ID NO: 98 - protein, 11 aa, synthetic construct
  REGION 1..11: note = Description of Artificial Sequence: Synthetic peptide
RASQSISSWLA

SEQ ID NO: 99 - protein, 7 aa, synthetic construct
  REGION 1..7: note = Description of Artificial Sequence: Synthetic peptide
KASSLES

SEQ ID NO: 100 - protein, 10 aa, synthetic construct
  REGION 1..10: note = Description of Artificial Sequence: Synthetic peptide
QQFQSLPPFT

SEQ ID NO: 101 - protein, 6 aa, synthetic construct
  REGION 1..6: note = Description of Artificial Sequence: Synthetic peptide
DVYGIS

SEQ ID NO: 102 - protein, 13 aa, synthetic construct
  REGION 1..13: note = Description of Artificial Sequence: Synthetic peptide
WMGWIAPYNGNTN

SEQ ID NO: 103 - protein, 15 aa, synthetic construct
  REGION 1..15: note = Description of Artificial Sequence: Synthetic peptide
ARDAGTYSPFGYGMD

SEQ ID NO: 104 - protein, 7 aa, synthetic construct
  REGION 1..7: note = Description of Artificial Sequence: Synthetic peptide
SSWLAWY

SEQ ID NO: 105 - protein, 10 aa, synthetic construct
  REGION 1..10: note = Description of Artificial Sequence: Synthetic peptide
LLIYKASSLE

SEQ ID NO: 106 - protein, 9 aa, synthetic construct
  REGION 1..9: note = Description of Artificial Sequence: Synthetic peptide
QQFQSLPPF

SEQ ID NO: 107 - protein, 8 aa, synthetic construct
  REGION 1..8: note = Description of Artificial Sequence: Synthetic peptide
GYTFDVYG

SEQ ID NO: 108 - protein, 8 aa, synthetic construct
  REGION 1..8: note = Description of Artificial Sequence: Synthetic peptide
IAPYNGNT

SEQ ID NO: 109 - protein, 16 aa, synthetic construct
  REGION 1..16: note = Description of Artificial Sequence: Synthetic peptide
ARDAGTYSPFGTGMDV

SEQ ID NO: 110 - protein, 6 aa, synthetic construct
  REGION 1..6: note = Description of Artificial Sequence: Synthetic peptide
QSISSW

SEQ ID NO: 111 - skipped

SEQ ID NO: 112 - protein, 10 aa, synthetic construct
  REGION 1..10: note = Description of Artificial Sequence: Synthetic peptide
QQFQSLPPFT

SEQ ID NO: 113 - protein, 123 aa, synthetic construct
  REGION 1..123: note = Description of Artificial Sequence: Synthetic polypeptide
QVQLVQSGAEVKKPGASVKVSCKASGYTFDVYGISWVRQAPGQGLEWMGWIAPYNGNTNYAQKLQGRVTMTTDTSTSTAYMELRSLRSDDTAVYYCARDAGTYSPFGYGMDVWGQGTTVTVSS

SEQ ID NO: 114 - protein, 108 aa, synthetic construct
  REGION 1..108: note = Description of Artificial Sequence: Synthetic polypeptide
DIQMTQSPSTLSASVGDRVTITCRASQSISSWLAWYQQKPGKAPKLLIYKASSLESGVPSRFSGSGSGTEFTLTISSLQPDDFATYYCQQFQSLPPFTFGGGTKVEIK

SEQ ID NO: 115 - protein, 10 aa, synthetic construct
  REGION 1..10: note = Description of Artificial Sequence: Synthetic peptide
GYTFDVYGIS

SEQ ID NO: 116 - protein, 17 aa, synthetic construct
  REGION 1..17: note = Description of Artificial Sequence: Synthetic peptide
WIAPYSGNTNYAQKLQG

SEQ ID NO: 117 - protein, 14 aa, synthetic construct
  REGION 1..14: note = Description of Artificial Sequence: Synthetic peptide
DAGTYSPFGYGMDV

SEQ ID NO: 118 - protein, 11 aa, synthetic construct
  REGION 1..11: note = Description of Artificial Sequence: Synthetic peptide
QASQSINNWLA

SEQ ID NO: 119 - protein, 7 aa, synthetic construct
  REGION 1..7: note = Description of Artificial Sequence: Synthetic peptide
KAYNLES

SEQ ID NO: 120 - protein, 10 aa, synthetic construct
  REGION 1..10: note = Description of Artificial Sequence: Synthetic peptide
QLFQSLPPFT

SEQ ID NO: 121 - protein, 5 aa, synthetic construct
  REGION 1..5: note = Description of Artificial Sequence: Synthetic peptide
VYGIS

SEQ ID NO: 122 - protein, 17 aa, synthetic construct
  REGION 1..17: note = Description of Artificial Sequence: Synthetic peptide
WIAPYSGNTNYAQKLQG

SEQ ID NO: 123 - protein, 14 aa, synthetic construct
  REGION 1..14: note = Description of Artificial Sequence: Synthetic peptide
DAGTYSPFGYGMDV

SEQ ID NO: 124 - protein, 11 aa, synthetic construct
  REGION 1..11: note = Description of Artificial Sequence: Synthetic peptide
QASQSINNWLA

SEQ ID NO: 125 - protein, 7 aa, synthetic construct
  REGION 1..7: note = Description of Artificial Sequence: Synthetic peptide
KAYNLES

SEQ ID NO: 126 - protein, 10 aa, synthetic construct
  REGION 1..10: note = Description of Artificial Sequence: Synthetic peptide
QLFQSLPPFT

SEQ ID NO: 127 - protein, 7 aa, synthetic construct
  REGION 1..7: note = Description of Artificial Sequence: Synthetic peptide
GYTFDVY

SEQ ID NO: 128 - protein, 4 aa, synthetic construct
  REGION 1..4: note = Description of Artificial Sequence: Synthetic peptide
PYSG

SEQ ID NO: 129 - protein, 12 aa, synthetic construct
  REGION 1..12: note = Description of Artificial Sequence: Synthetic peptide
AGTYSPFGYGMD

SEQ ID NO: 130 - protein, 7 aa, synthetic construct
  REGION 1..7: note = Description of Artificial Sequence: Synthetic peptide
SQSINNW

SEQ ID NO: 131 - skipped

SEQ ID NO: 132 - protein, 7 aa, synthetic construct
  REGION 1..7: note = Description of Artificial Sequence: Synthetic peptide
FQSLPPF

SEQ ID NO: 133 - protein, 10 aa, synthetic construct
  REGION 1..10: note = Description of Artificial Sequence: Synthetic peptide
GYTFDVYGIS

SEQ ID NO: 134 - protein, 10 aa, synthetic construct
  REGION 1..10: note = Description of Artificial Sequence: Synthetic peptide
WIAPYSGNTN

SEQ ID NO: 135 - protein, 14 aa, synthetic construct
  REGION 1..14: note = Description of Artificial Sequence: Synthetic peptide
DAGTYSPFGYGMDV

SEQ ID NO: 136 - protein, 11 aa, synthetic construct
  REGION 1..11: note = Description of Artificial Sequence: Synthetic peptide
QASQSINNWLA

SEQ ID NO: 137 - protein, 7 aa, synthetic construct
  REGION 1..7: note = Description of Artificial Sequence: Synthetic peptide
KAYNLES

SEQ ID NO: 138 - protein, 10 aa, synthetic construct
  REGION 1..10: note = Description of Artificial Sequence: Synthetic peptide
QLFQSLPPFT

SEQ ID NO: 139 - protein, 6 aa, synthetic construct
  REGION 1..6: note = Description of Artificial Sequence: Synthetic peptide
DVYGIS

SEQ ID NO: 140 - protein, 13 aa, synthetic construct
  REGION 1..13: note = Description of Artificial Sequence: Synthetic peptide
WMGWIAPYSGNTN

SEQ ID NO: 141 - protein, 15 aa, synthetic construct
  REGION 1..15: note = Description of Artificial Sequence: Synthetic peptide
ARDAGTYSPFGYGMD

SEQ ID NO: 142 - protein, 7 aa, synthetic construct
  REGION 1..7: note = Description of Artificial Sequence: Synthetic peptide
NNWLAWY

SEQ ID NO: 143 - protein, 10 aa, synthetic construct
  REGION 1..10: note = Description of Artificial Sequence: Synthetic peptide
LLIYKAYNLE

SEQ ID NO: 144 - protein, 9 aa, synthetic construct
  REGION 1..9: note = Description of Artificial Sequence: Synthetic peptide
QLFQSLPPF

SEQ ID NO: 145 - protein, 8 aa, synthetic construct
  REGION 1..8: note = Description of Artificial Sequence: Synthetic peptide
GYTFDVYG

SEQ ID NO: 146 - protein, 8 aa, synthetic construct
  REGION 1..8: note = Description of Artificial Sequence: Synthetic peptide
IAPYSGNT

SEQ ID NO: 147 - protein, 16 aa, synthetic construct
  REGION 1..16: note = Description of Artificial Sequence: Synthetic peptide
ARDAGTYSPFGTGMDV

SEQ ID NO: 148 - protein, 6 aa, synthetic construct
  REGION 1..6: note = Description of Artificial Sequence: Synthetic peptide
QSINNW

SEQ ID NO: 149 - skipped

SEQ ID NO: 150 - protein, 10 aa, synthetic construct
  REGION 1..10: note = Description of Artificial Sequence: Synthetic peptide
QLFQSLPPFT

SEQ ID NO: 151 - protein, 123 aa, synthetic construct
  REGION 1..123: note = Description of Artificial Sequence: Synthetic polypeptide
QVQLVQSGAEVKKPGASVKVSCKASGYTFDVYGISWVRQAPGQGLEWMGWIAPYSGNTNYAQKLQGRVTMTTDTSTSTAYMELRSLRSDDTAVYYCARDAGTYSPFGYGMDVWGQGTTVTVSS

SEQ ID NO: 152 - protein, 108 aa, synthetic construct
  REGION 1..108: note = Description of Artificial Sequence: Synthetic polypeptide
DIQMTQSPSTLSASVGDRVTITCQASQSINNWLAWYQQKPGKAPKLLIYKAYNLESGVPSRFSGSGSGTEFTLTISSLQPDDFATYYCQLFQSLPPFTFGGGTKVEIK

SEQ ID NO: 153 - protein, 10 aa, synthetic construct
  REGION 1..10: note = Description of Artificial Sequence: Synthetic peptide
GYTFDVYGIS

SEQ ID NO: 154 - protein, 17 aa, synthetic construct
  REGION 1..17: note = Description of Artificial Sequence: Synthetic peptide
WIAPYSGNTNYAQKLQG

SEQ ID NO: 155 - protein, 14 aa, synthetic construct
  REGION 1..14: note = Description of Artificial Sequence: Synthetic peptide
DAGTYSPFGYGMDV

SEQ ID NO: 156 - protein, 11 aa, synthetic construct
  REGION 1..11: note = Description of Artificial Sequence: Synthetic peptide
RASESISNWLA

SEQ ID NO: 157 - protein, 7 aa, synthetic construct
  REGION 1..7: note = Description of Artificial Sequence: Synthetic peptide
KAYSLEY

SEQ ID NO: 158 - protein, 10 aa, synthetic construct
  REGION 1..10: note = Description of Artificial Sequence: Synthetic peptide
QQFQKLPPFT

SEQ ID NO: 159 - protein, 5 aa, synthetic construct
  REGION 1..5: note = Description of Artificial Sequence: Synthetic peptide
VYGIS

SEQ ID NO: 160 - protein, 17 aa, synthetic construct
  REGION 1..17: note = Description of Artificial Sequence: Synthetic peptide
WIAPYSGNTNYAQKLQG

SEQ ID NO: 161 - protein, 14 aa, synthetic construct
  REGION 1..14: note = Description of Artificial Sequence: Synthetic peptide
DAGTYSPFGYGMDV

SEQ ID NO: 162 - protein, 11 aa, synthetic construct
  REGION 1..11: note = Description of Artificial Sequence: Synthetic peptide
RASESISNWLA

SEQ ID NO: 163 - protein, 7 aa, synthetic construct
  REGION 1..7: note = Description of Artificial Sequence: Synthetic peptide
KAYSLEY

SEQ ID NO: 164 - protein, 10 aa, synthetic construct
  REGION 1..10: note = Description of Artificial Sequence: Synthetic peptide
QQFQKLPPFT

SEQ ID NO: 165 - protein, 7 aa, synthetic construct
  REGION 1..7: note = Description of Artificial Sequence: Synthetic peptide
GYTFDVY

SEQ ID NO: 166 - protein, 4 aa, synthetic construct
  REGION 1..4: note = Description of Artificial Sequence: Synthetic peptide
PYSG

SEQ ID NO: 167 - protein, 12 aa, synthetic construct
  REGION 1..12: note = Description of Artificial Sequence: Synthetic peptide
AGTYSPFGYGMD

SEQ ID NO: 168 - protein, 7 aa, synthetic construct
  REGION 1..7: note = Description of Artificial Sequence: Synthetic peptide
SESISNW

SEQ ID NO: 169 - skipped

SEQ ID NO: 170 - protein, 7 aa, synthetic construct
  REGION 1..7: note = Description of Artificial Sequence: Synthetic peptide
FQKLPPF

SEQ ID NO: 171 - protein, 10 aa, synthetic construct
  REGION 1..10: note = Description of Artificial Sequence: Synthetic peptide
GYTFDVYGIS

SEQ ID NO: 172 - protein, 10 aa, synthetic construct
  REGION 1..10: note = Description of Artificial Sequence: Synthetic peptide
WIAPYSGNTN

SEQ ID NO: 173 - protein, 14 aa, synthetic construct
  REGION 1..14: note = Description of Artificial Sequence: Synthetic peptide
DAGTYSPFGYGMDV

SEQ ID NO: 174 - protein, 11 aa, synthetic construct
  REGION 1..11: note = Description of Artificial Sequence: Synthetic peptide
RASESISNWLA

SEQ ID NO: 175 - protein, 7 aa, synthetic construct
  REGION 1..7: note = Description of Artificial Sequence: Synthetic peptide
KAYSLEY

SEQ ID NO: 176 - protein, 10 aa, synthetic construct
  REGION 1..10: note = Description of Artificial Sequence: Synthetic peptide
QQFQKLPPFT

SEQ ID NO: 177 - protein, 6 aa, synthetic construct
  REGION 1..6: note = Description of Artificial Sequence: Synthetic peptide
DVYGIS

SEQ ID NO: 178 - protein, 13 aa, synthetic construct
  REGION 1..13: note = Description of Artificial Sequence: Synthetic peptide
WMGWIAPYSGNTN

SEQ ID NO: 179 - protein, 15 aa, synthetic construct
  REGION 1..15: note = Description of Artificial Sequence: Synthetic peptide
ARDAGTYSPFGYGMD

SEQ ID NO: 180 - protein, 7 aa, synthetic construct
  REGION 1..7: note = Description of Artificial Sequence: Synthetic peptide
SNWLAWY

SEQ ID NO: 181 - protein, 10 aa, synthetic construct
  REGION 1..10: note = Description of Artificial Sequence: Synthetic peptide
LLIYKAYSLE

SEQ ID NO: 182 - protein, 9 aa, synthetic construct
  REGION 1..9: note = Description of Artificial Sequence: Synthetic peptide
QQFQKLPPF

SEQ ID NO: 183 - protein, 8 aa, synthetic construct
  REGION 1..8: note = Description of Artificial Sequence: Synthetic peptide
GYTFDVYG

SEQ ID NO: 184 - protein, 8 aa, synthetic construct
  REGION 1..8: note = Description of Artificial Sequence: Synthetic peptide
IAPYSGNT

SEQ ID NO: 185 - protein, 16 aa, synthetic construct
  REGION 1..16: note = Description of Artificial Sequence: Synthetic peptide
ARDAGTYSPFGTGMDV

SEQ ID NO: 186 - protein, 6 aa, synthetic construct
  REGION 1..6: note = Description of Artificial Sequence: Synthetic peptide
ESISNW

SEQ ID NO: 187 - skipped

SEQ ID NO: 188 - protein, 10 aa, synthetic construct
  REGION 1..10: note = Description of Artificial Sequence: Synthetic peptide
QQFQKLPPFT

SEQ ID NO: 189 - protein, 123 aa, synthetic construct; identical to SEQ ID NO: 151
  REGION 1..123: note = Description of Artificial Sequence: Synthetic polypeptide

SEQ ID NO: 190 - protein, 108 aa, synthetic construct
  REGION 1..108: note = Description of Artificial Sequence: Synthetic polypeptide
DIQMTQSPSTLSASVGDRVTITCRASESISNWLAWYQQKPGKAPKLLIYKAYSLEYGVPSRFSGSGSGTEFTLTISSLQPDDFATYYCQQFQKLPPFTFGGGTKVEIK

SEQ ID NO: 191 - protein, 10 aa, synthetic construct
  REGION 1..10: note = Description of Artificial Sequence: Synthetic peptide
GYTFRSYGIS

SEQ ID NO: 192 - protein, 17 aa, synthetic construct
  REGION 1..17: note = Description of Artificial Sequence: Synthetic peptide
WVAPYNGNTNYAQKLQG

SEQ ID NO: 193 - protein, 14 aa, synthetic construct
  REGION 1..14: note = Description of Artificial Sequence: Synthetic peptide
DAGTYSPYGYGMDV

SEQ ID NO: 194 - protein, 11 aa, synthetic construct
  REGION 1..11: note = Description of Artificial Sequence: Synthetic peptide
RASQSISSWLA

SEQ ID NO: 195 - protein, 7 aa, synthetic construct
  REGION 1..7: note = Description of Artificial Sequence: Synthetic peptide
KASSLES

SEQ ID NO: 196 - protein, 10 aa, synthetic construct
  REGION 1..10: note = Description of Artificial Sequence: Synthetic peptide
QQFQSLPPFT

SEQ ID NO: 197 - protein, 5 aa, synthetic construct
  REGION 1..5: note = Description of Artificial Sequence: Synthetic peptide
SYGIS

SEQ ID NO: 198 - protein, 17 aa, synthetic construct
  REGION 1..17: note = Description of Artificial Sequence: Synthetic peptide
WVAPYNGNTNYAQKLQG

SEQ ID NO: 199 - protein, 14 aa, synthetic construct
  REGION 1..14: note = Description of Artificial Sequence: Synthetic peptide
DAGTYSPYGYGMDV

SEQ ID NO: 200 - protein, 11 aa, synthetic construct
  REGION 1..11: note = Description of Artificial Sequence: Synthetic peptide
RASQSISSWLA

SEQ ID NO: 201 - protein, 7 aa, synthetic construct
  REGION 1..7: note = Description of Artificial Sequence: Synthetic peptide
KASSLES

SEQ ID NO: 202 - protein, 10 aa, synthetic construct
  REGION 1..10: note = Description of Artificial Sequence: Synthetic peptide
QQFQSLPPFT

SEQ ID NO: 203 - protein, 7 aa, synthetic construct
  REGION 1..7: note = Description of Artificial Sequence: Synthetic peptide
GYTFRSY

SEQ ID NO: 204 - protein, 4 aa, synthetic construct
  REGION 1..4: note = Description of Artificial Sequence: Synthetic peptide
PYNG

SEQ ID NO: 205 - protein, 12 aa, synthetic construct
  REGION 1..12: note = Description of Artificial Sequence: Synthetic peptide
AGTYSPYGYGMD

SEQ ID NO: 206 - protein, 7 aa, synthetic construct
  REGION 1..7: note = Description of Artificial Sequence: Synthetic peptide
SQSISSW

SEQ ID NO: 207 - skipped

SEQ ID NO: 208 - protein, 7 aa, synthetic construct
  REGION 1..7: note = Description of Artificial Sequence: Synthetic peptide
FQSLPPF

SEQ ID NO: 209 - protein, 10 aa, synthetic construct
  REGION 1..10: note = Description of Artificial Sequence: Synthetic peptide
GYTFRSYGIS

SEQ ID NO: 210 - protein, 10 aa, synthetic construct
  REGION 1..10: note = Description of Artificial Sequence: Synthetic peptide
WVAPYNGNTN

SEQ ID NO: 211 - protein, 14 aa, synthetic construct
  REGION 1..14: note = Description of Artificial Sequence: Synthetic peptide
DAGTYSPYGYGMDV

SEQ ID NO: 212 - protein, 11 aa, synthetic construct
  REGION 1..11: note = Description of Artificial Sequence: Synthetic peptide
RASQSISSWLA

SEQ ID NO: 213 - protein, 7 aa, synthetic construct
  REGION 1..7: note = Description of Artificial Sequence: Synthetic peptide
KASSLES

SEQ ID NO: 214 - protein, 10 aa, synthetic construct
  REGION 1..10: note = Description of Artificial Sequence: Synthetic peptide
QQFQSLPPFT

SEQ ID NO: 215 - protein, 6 aa, synthetic construct
  REGION 1..6: note = Description of Artificial Sequence: Synthetic peptide
RSYGIS

SEQ ID NO: 216 - protein, 13 aa, synthetic construct
  REGION 1..13: note = Description of Artificial Sequence: Synthetic peptide
WMGWVAPYNGNTN

SEQ ID NO: 217 - protein, 15 aa, synthetic construct
  REGION 1..15: note = Description of Artificial Sequence: Synthetic peptide
ARDAGTYSPYGYGMD

SEQ ID NO: 218 - protein, 7 aa, synthetic construct
  REGION 1..7: note = Description of Artificial Sequence: Synthetic peptide
SSWLAWY

SEQ ID NO: 219 - protein, 10 aa, synthetic construct
  REGION 1..10: note = Description of Artificial Sequence: Synthetic peptide
LLIYKASSLE

SEQ ID NO: 220 - protein, 9 aa, synthetic construct
  REGION 1..9: note = Description of Artificial Sequence: Synthetic peptide
QQFQSLPPF

SEQ ID NO: 221 - protein, 8 aa, synthetic construct
  REGION 1..8: note = Description of Artificial Sequence: Synthetic peptide
GYTFRSYG

SEQ ID NO: 222 - protein, 8 aa, synthetic construct
  REGION 1..8: note = Description of Artificial Sequence: Synthetic peptide
VAPYNGNT

SEQ ID NO: 223 - protein, 16 aa, synthetic construct
  REGION 1..16: note = Description of Artificial Sequence: Synthetic peptide
ARDAGTYSPYGYGMDV

SEQ ID NO: 224 - protein, 6 aa, synthetic construct
  REGION 1..6: note = Description of Artificial Sequence: Synthetic peptide
QSISSW

SEQ ID NO: 225 - skipped

SEQ ID NO: 226 - protein, 10 aa, synthetic construct
  REGION 1..10: note = Description of Artificial Sequence: Synthetic peptide
QQFQSLPPFT

SEQ ID NO: 227 - protein, 123 aa, synthetic construct
  REGION 1..123: note = Description of Artificial Sequence: Synthetic polypeptide
QVQLVQSGAEVKKPGASVKVSCKASGYTFRSYGISWVRQAPGQGLEWMGWVAPYNGNTNYAQKLQGRVTMTTDTSTSTAYMELRSLRSDDTAVYYCARDAGTYSPYGYGMDVWGQGTTVTVSS

SEQ ID NO: 228 - protein, 108 aa, synthetic construct; identical to SEQ ID NO: 114
  REGION 1..108: note = Description of Artificial Sequence: Synthetic polypeptide

SEQ ID NO: 229 - protein, 10 aa, synthetic construct
  REGION 1..10: note = Description of Artificial Sequence: Synthetic peptide
GYTFRSYGIS

SEQ ID NO: 230 - protein, 17 aa, synthetic construct
  REGION 1..17: note = Description of Artificial Sequence: Synthetic peptide
WVAPYSGNTNYAQKLQG

SEQ ID NO: 231 - protein, 14 aa, synthetic construct
  REGION 1..14: note = Description of Artificial Sequence: Synthetic peptide
DAGTYSPYGYGMDV

SEQ ID NO: 232 - protein, 11 aa, synthetic construct
  REGION 1..11: note = Description of Artificial Sequence: Synthetic peptide
RASHSIDSWLA

SEQ ID NO: 233 - protein, 7 aa, synthetic construct
  REGION 1..7: note = Description of Artificial Sequence: Synthetic peptide
KASYLES

SEQ ID NO: 234 - protein, 10 aa, synthetic construct
  REGION 1..10: note = Description of Artificial Sequence: Synthetic peptide
QLFQSLPPFT

SEQ ID NO: 235 - protein, 5 aa, synthetic construct
  REGION 1..5: note = Description of Artificial Sequence: Synthetic peptide
SYGIS

SEQ ID NO: 236 - protein, 17 aa, synthetic construct
  REGION 1..17: note = Description of Artificial Sequence: Synthetic peptide
WVAPYSGNTNYAQKLQG

SEQ ID NO: 237 - protein, 14 aa, synthetic construct
  REGION 1..14: note = Description of Artificial Sequence: Synthetic peptide
DAGTYSPYGYGMDV

SEQ ID NO: 238 - protein, 11 aa, synthetic construct
  REGION 1..11: note = Description of Artificial Sequence: Synthetic peptide
RASHSIDSWLA

SEQ ID NO: 239 - protein, 7 aa, synthetic construct
  REGION 1..7: note = Description of Artificial Sequence: Synthetic peptide
KASYLES

SEQ ID NO: 240 - protein, 10 aa, synthetic construct
  REGION 1..10: note = Description of Artificial Sequence: Synthetic peptide
QLFQSLPPFT

SEQ ID NO: 241 - protein, 7 aa, synthetic construct
  REGION 1..7: note = Description of Artificial Sequence: Synthetic peptide
GYTFRSY

SEQ ID NO: 242 - protein, 4 aa, synthetic construct
  REGION 1..4: note = Description of Artificial Sequence: Synthetic peptide
PYSG

SEQ ID NO: 243 - protein, 12 aa, synthetic construct
  REGION 1..12: note = Description of Artificial Sequence: Synthetic peptide
AGTYSPYGYGMD

SEQ ID NO: 244 - protein, 7 aa, synthetic construct
  REGION 1..7: note = Description of Artificial Sequence: Synthetic peptide
SHSIDSW

SEQ ID NO: 245 - skipped

SEQ ID NO: 246 - protein, 7 aa, synthetic construct
  REGION 1..7: note = Description of Artificial Sequence: Synthetic peptide
FQSLPPF

SEQ ID NO: 247 - protein, 10 aa, synthetic construct
  REGION 1..10: note = Description of Artificial Sequence: Synthetic peptide
GYTFRSYGIS

SEQ ID NO: 248 - protein, 10 aa, synthetic construct
  REGION 1..10: note = Description of Artificial Sequence: Synthetic peptide
WVAPYSGNTN

SEQ ID NO: 249 - protein, 14 aa, synthetic construct
  REGION 1..14: note = Description of Artificial Sequence: Synthetic peptide
DAGTYSPYGYGMDV

SEQ ID NO: 250 - protein, 11 aa, synthetic construct
  REGION 1..11: note = Description of Artificial Sequence: Synthetic peptide
RASHSIDSWLA

SEQ ID NO: 251 - protein, 7 aa, synthetic construct
  REGION 1..7: note = Description of Artificial Sequence: Synthetic peptide
KASYLES

SEQ ID NO: 252 - protein, 10 aa, synthetic construct
  REGION 1..10: note = Description of Artificial Sequence: Synthetic peptide
QLFQSLPPFT

SEQ ID NO: 253 - protein, 6 aa, synthetic construct
  REGION 1..6: note = Description of Artificial Sequence: Synthetic peptide
RSYGIS

SEQ ID NO: 254 - protein, 13 aa, synthetic construct
  REGION 1..13: note = Description of Artificial Sequence: Synthetic peptide
WMGWVAPYSGNTN

SEQ ID NO: 255 - protein, 15 aa, synthetic construct
  REGION 1..15: note = Description of Artificial Sequence: Synthetic peptide
ARDAGTYSPYGYGMD

SEQ ID NO: 256 - protein, 7 aa, synthetic construct
  REGION 1..7: note = Description of Artificial Sequence: Synthetic peptide
DSWLAWY

SEQ ID NO: 257 - protein, 10 aa, synthetic construct
  REGION 1..10: note = Description of Artificial Sequence: Synthetic peptide
LLIYKASYLE

SEQ ID NO: 258 - protein, 9 aa, synthetic construct
  REGION 1..9: note = Description of Artificial Sequence: Synthetic peptide
QLFQSLPPF

SEQ ID NO: 259 - protein, 8 aa, synthetic construct
  REGION 1..8: note = Description of Artificial Sequence: Synthetic peptide
GYTFRSYG

SEQ ID NO: 260 - protein, 8 aa, synthetic construct
  REGION 1..8: note = Description of Artificial Sequence: Synthetic peptide
VAPYSGNT

SEQ ID NO: 261 - protein, 16 aa, synthetic construct
  REGION 1..16: note = Description of Artificial Sequence: Synthetic peptide
ARDAGTYSPYGYGMDV

SEQ ID NO: 262 - protein, 6 aa, synthetic construct
  REGION 1..6: note = Description of Artificial Sequence: Synthetic peptide
HSIDSW

SEQ ID NO: 263 - skipped

SEQ ID NO: 264 - protein, 10 aa, synthetic construct
  REGION 1..10: note = Description of Artificial Sequence: Synthetic peptide
QLFQSLPPFT

SEQ ID NO: 265 - protein, 123 aa, synthetic construct
  REGION 1..123: note = Description of Artificial Sequence: Synthetic polypeptide
QVQLVQSGAEVKKPGASVKVSCKASGYTFRSYGISWVRQAPGQGLEWMGWVAPYSGNTNYAQKLQGRVTMTTDTSTSTAYMELRSLRSDDTAVYYCARDAGTYSPYGYGMDVWGQGTTVTVSS

SEQ ID NO: 266 - protein, 108 aa, synthetic construct
  REGION 1..108: note = Description of Artificial Sequence: Synthetic polypeptide
DIQMTQSPSTLSASVGDRVTITCRASHSIDSWLAWYQQKPGKAPKLLIYKASYLESGVPSRFSGSGSGTEFTLTISSLQPDDFATYYCQLFQSLPPFTFGGGTKVEIK

SEQ ID NO: 267 - protein, 10 aa, synthetic construct
  REGION 1..10: note = Description of Artificial Sequence: Synthetic peptide
GYTFRSYGIS

SEQ ID NO: 268 - protein, 17 aa, synthetic construct
  REGION 1..17: note = Description of Artificial Sequence: Synthetic peptide
WVAPYSGNTNYAQKLQG

SEQ ID NO: 269 - protein, 14 aa, synthetic construct
  REGION 1..14: note = Description of Artificial Sequence: Synthetic peptide
DAGTYSPYGYGMDV

SEQ ID NO: 270 - protein, 11 aa, synthetic construct
  REGION 1..11: note = Description of Artificial Sequence: Synthetic peptide
QASQSIDSWLA

SEQ ID NO: 271 - protein, 7 aa, synthetic construct
  REGION 1..7: note = Description of Artificial Sequence: Synthetic peptide
SASYLES

SEQ ID NO: 272 - protein, 10 aa, synthetic construct
  REGION 1..10: note = Description of Artificial Sequence: Synthetic peptide
QRFQSLPPFT

SEQ ID NO: 273 - protein, 5 aa, synthetic construct
  REGION 1..5: note = Description of Artificial Sequence: Synthetic peptide
SYGIS

SEQ ID NO: 274 - protein, 17 aa, synthetic construct
  REGION 1..17: note = Description of Artificial Sequence: Synthetic peptide
WVAPYSGNTNYAQKLQG

SEQ ID NO: 275 - protein, 14 aa, synthetic construct
  REGION 1..14: note = Description of Artificial Sequence: Synthetic peptide
DAGTYSPYGYGMDV

SEQ ID NO: 276 - protein, 11 aa, synthetic construct
  REGION 1..11: note = Description of Artificial Sequence: Synthetic peptide
QASQSIDSWLA

SEQ ID NO: 277 - protein, 7 aa, synthetic construct
  REGION 1..7: note = Description of Artificial Sequence: Synthetic peptide
SASYLES

SEQ ID NO: 278 - protein, 10 aa, synthetic construct
  REGION 1..10: note = Description of Artificial Sequence: Synthetic peptide
QRFQSLPPFT

SEQ ID NO: 279 - protein, 7 aa, synthetic construct
  REGION 1..7: note = Description of Artificial Sequence: Synthetic peptide
GYTFRSY

SEQ ID NO: 280 - protein, 4 aa, synthetic construct
  REGION 1..4: note = Description of Artificial Sequence: Synthetic peptide
PYSG

SEQ ID NO: 281 - protein, 12 aa, synthetic construct
  REGION 1..12: note = Description of Artificial Sequence: Synthetic peptide
AGTYSPYGYGMD

SEQ ID NO: 282 - protein, 7 aa, synthetic construct
  REGION 1..7: note = Description of Artificial Sequence: Synthetic peptide
SQSIDSW

SEQ ID NO: 283 - skipped

SEQ ID NO: 284 - protein, 7 aa, synthetic construct
  REGION 1..7: note = Description of Artificial Sequence: Synthetic peptide
FQSLPPF

SEQ ID NO: 285 - protein, 10 aa, synthetic construct
  REGION 1..10: note = Description of Artificial Sequence: Synthetic peptide
GYTFRSYGIS

SEQ ID NO: 286 - protein, 10 aa, synthetic construct
  REGION 1..10: note = Description of Artificial Sequence: Synthetic peptide
WVAPYSGNTN

SEQ ID NO: 287 - protein, 14 aa, synthetic construct
  REGION 1..14: note = Description of Artificial Sequence: Synthetic peptide
DAGTYSPYGYGMDV

SEQ ID NO: 288 - protein, 11 aa, synthetic construct
  REGION 1..11: note = Description of Artificial Sequence: Synthetic peptide
QASQSIDSWLA

SEQ ID NO: 289 - protein, 7 aa, synthetic construct
  REGION 1..7: note = Description of Artificial Sequence: Synthetic peptide
SASYLES

SEQ ID NO: 290 - protein, 10 aa, synthetic construct
  REGION 1..10: note = Description of Artificial Sequence: Synthetic peptide
QRFQSLPPFT

SEQ ID NO: 291 - protein, 6 aa, synthetic construct
  REGION 1..6: note = Description of Artificial Sequence: Synthetic peptide
RSYGIS

SEQ ID NO: 292 - protein, 13 aa, synthetic construct
  REGION 1..13: note = Description of Artificial Sequence: Synthetic peptide
WMGWVAPYSGNTN

SEQ ID NO: 293 - protein, 15 aa, synthetic construct
  REGION 1..15: note = Description of Artificial Sequence: Synthetic peptide
ARDAGTYSPYGYGMD

SEQ ID NO: 294 - protein, 7 aa, synthetic construct
  REGION 1..7: note = Description of Artificial Sequence: Synthetic peptide
DSWLAWY

SEQ ID NO: 295 - protein, 10 aa, synthetic construct
  REGION 1..10: note = Description of Artificial Sequence: Synthetic peptide
LLIYSASYLE

SEQ ID NO: 296 - protein, 9 aa, synthetic construct
  REGION 1..9: note = Description of Artificial Sequence: Synthetic peptide
QRFQSLPPF

SEQ ID NO: 297 - protein, 8 aa, synthetic construct
  REGION 1..8: note = Description of Artificial Sequence: Synthetic peptide
GYTFRSYG

SEQ ID NO: 298 - protein, 8 aa, synthetic construct
  REGION 1..8: note = Description of Artificial Sequence: Synthetic peptide
VAPYSGNT

SEQ ID NO: 299 - protein, 16 aa, synthetic construct
  REGION 1..16: note = Description of Artificial Sequence: Synthetic peptide
ARDAGTYSPYGYGMDV

SEQ ID NO: 300 - protein, 6 aa, synthetic construct
  REGION 1..6: note = Description of Artificial Sequence: Synthetic peptide
QSIDSW

SEQ ID NO: 301 - skipped

SEQ ID NO: 302 - protein, 10 aa, synthetic construct
  REGION 1..10: note = Description of Artificial Sequence: Synthetic peptide
QRFQSLPPFT

SEQ ID NO: 303 - protein, 123 aa, synthetic construct; identical to SEQ ID NO: 265
  REGION 1..123: note = Description of Artificial Sequence: Synthetic polypeptide

SEQ ID NO: 304 - protein, 108 aa, synthetic construct
  REGION 1..108: note = Description of Artificial Sequence: Synthetic polypeptide
DIQMTQSPSTLSASVGDRVTITCQASQSIDSWLAWYQQKPGKAPKLLIYSASYLESGVPSRFSGSGSGTEFTLTISSLQPDDFATYYCQRFQSLPPFTFGGGTKVEIK

SEQ ID NO: 305 - protein, 10 aa, synthetic construct
  REGION 1..10: note = Description of Artificial Sequence: Synthetic peptide
GFTFHSRGMH

SEQ ID NO: 306 - protein, 17 aa, synthetic construct
  REGION 1..17: note = Description of Artificial Sequence: Synthetic peptide
VITYDGINKYYADSVEG

SEQ ID NO: 307 - protein, 10 aa, synthetic construct
  REGION 1..10: note = Description of Artificial Sequence: Synthetic peptide
DGVYYGVYDY

SEQ ID NO: 308 - protein, 17 aa, synthetic construct
  REGION 1..17: note = Description of Artificial Sequence: Synthetic peptide
KSSQSVLFSSNNKNYLA

SEQ ID NO: 309 - protein, 7 aa, synthetic construct
  REGION 1..7: note = Description of Artificial Sequence: Synthetic peptide
WASTRES

SEQ ID NO: 310 - protein, 9 aa, synthetic construct
  REGION 1..9: note = Description of Artificial Sequence: Synthetic peptide
QQFHSYPLT

SEQ ID NO: 311 - protein, 5 aa, synthetic construct
  REGION 1..5: note = Description of Artificial Sequence: Synthetic peptide
SRGMH

SEQ ID NO: 312 - protein, 17 aa, synthetic construct
  REGION 1..17: note = Description of Artificial Sequence: Synthetic peptide
VITYDGINKYYADSVEG

SEQ ID NO: 313 - protein, 10 aa, synthetic construct
  REGION 1..10: note = Description of Artificial Sequence: Synthetic peptide
DGVYYGVYDY

SEQ ID NO: 314 - protein, 17 aa, synthetic construct
  REGION 1..17: note = Description of Artificial Sequence: Synthetic peptide
KSSQSVLFSSNNKNYLA

SEQ ID NO: 315 - protein, 7 aa, synthetic construct
  REGION 1..7: note = Description of Artificial Sequence: Synthetic peptide
WASTRES

SEQ ID NO: 316 - protein, 9 aa, synthetic construct
  REGION 1..9: note = Description of Artificial Sequence: Synthetic peptide
QQFHSYPLT

SEQ ID NO: 317 - protein, 7 aa, synthetic construct
  REGION 1..7: note = Description of Artificial Sequence: Synthetic peptide
GFTFHSR

SEQ ID NO: 318 - protein, 4 aa, synthetic construct
  REGION 1..4: note = Description of Artificial Sequence: Synthetic peptide
YDGI

SEQ ID NO: 319 - protein, 8 aa, synthetic construct
  REGION 1..8: note = Description of Artificial Sequence: Synthetic peptide
GVYYGVYD

SEQ ID NO: 320 - protein, 13 aa, synthetic construct
  REGION 1..13: note = Description of Artificial Sequence: Synthetic peptide
SQSVLFSSNNKNY

SEQ ID NO: 321 - skipped

SEQ ID NO: 322 - protein, 6 aa, synthetic construct
  REGION 1..6: note = Description of Artificial Sequence: Synthetic peptide
FHSYPL

SEQ ID NO: 323 - protein, 10 aa, synthetic construct
  REGION 1..10: note = Description of Artificial Sequence: Synthetic peptide
GFTFHSRGMH

SEQ ID NO: 324 - protein, 10 aa, synthetic construct
  REGION 1..10: note = Description of Artificial Sequence: Synthetic peptide
VITYDGINKY

SEQ ID NO: 325 - protein, 10 aa, synthetic construct
  REGION 1..10: note = Description of Artificial Sequence: Synthetic peptide
DGVYYGVYDY

SEQ ID NO: 326 - protein, 17 aa, synthetic construct
  REGION 1..17: note = Description of Artificial Sequence: Synthetic peptide
KSSQSVLFSSNNKNYLA

SEQ ID NO: 327 - protein, 7 aa, synthetic construct
  REGION 1..7: note = Description of Artificial Sequence: Synthetic peptide
WASTRES

SEQ ID NO: 328 - protein, 9 aa, synthetic construct
  REGION 1..9: note = Description of Artificial Sequence: Synthetic peptide
QQFHSYPLT

SEQ ID NO: 329 - protein, 6 aa, synthetic construct
  REGION 1..6: note = Description of Artificial Sequence: Synthetic peptide
HSRGMH

SEQ ID NO: 330 - protein, 13 aa, synthetic construct
  REGION 1..13: note = Description of Artificial Sequence: Synthetic peptide
WVAVITYDGINKY

SEQ ID NO: 331 - protein, 11 aa, synthetic construct
  REGION 1..11: note = Description of Artificial Sequence: Synthetic peptide
ARDGVYYGVYD

SEQ ID NO: 332 - protein, 13 aa, synthetic construct
  REGION 1..13: note = Description of Artificial Sequence: Synthetic peptide
LFSSNNKNYLAWY

SEQ ID NO: 333 - protein, 10 aa, synthetic construct
  REGION 1..10: note = Description of Artificial Sequence: Synthetic peptide
LLIYWASTRE

SEQ ID NO: 334 - protein, 8 aa, synthetic construct
  REGION 1..8: note = Description of Artificial Sequence: Synthetic peptide
QQFHSYPL

SEQ ID NO: 335 - protein, 8 aa, synthetic construct
  REGION 1..8: note = Description of Artificial Sequence: Synthetic peptide
GFTFHSRG

SEQ ID NO: 336 - protein, 8 aa, synthetic construct
  REGION 1..8: note = Description of Artificial Sequence: Synthetic peptide
ITYDGINK

SEQ ID NO: 337 - protein, 12 aa, synthetic construct
  REGION 1..12: note = Description of Artificial Sequence: Synthetic peptide
ARDGVYYGVYDY

SEQ ID NO: 338 - protein, 12 aa, synthetic construct
  REGION 1..12: note = Description of Artificial Sequence: Synthetic peptide
QSVLFSSNNKNY

SEQ ID NO: 339 - skipped

SEQ ID NO: 340 - protein, 9 aa, synthetic construct
  REGION 1..9: note = Description of Artificial Sequence: Synthetic peptide
QQFHSYPLT

SEQ ID NO: 341 - protein, 119 aa, synthetic construct
  REGION 1..119: note = Description of Artificial Sequence: Synthetic polypeptide
QVQLVESGGGVVQPGRSLRLSCAASGFTFHSRGMHWVRQAPGKGLEWVAVITYDGINKYYADSVEGRFTISRDNSKNTLYLQMNSLRAEDTAVYYCARDGVYYGVYDYWGQGTLVTVSS

SEQ ID NO: 342 - protein, 113 aa, synthetic construct
  REGION 1..113: note = Description of Artificial Sequence: Synthetic polypeptide
DIVMTQSPDSLAVSLGERATINCKSSQSVLFSSNNKNYLAWYQQKPGQPPKLLIYWASTRESGVPDRFSGSGSGTDFTLTISSLQAEDVAVYYCQQFHSYPLTFGGGTKVEIK

SEQ ID NO: 343 - protein, 10 aa, synthetic construct
  REGION 1..10: note = Description of Artificial Sequence: Synthetic peptide
GFTFRSYGMH

SEQ ID NO: 344 - protein, 17 aa, synthetic construct
  REGION 1..17: note = Description of Artificial Sequence: Synthetic peptide
VITYDGINKYYADSVEG

SEQ ID NO: 345 - protein, 10 aa, synthetic construct
  REGION 1..10: note = Description of Artificial Sequence: Synthetic peptide
DGVYYGVYDY

SEQ ID NO: 346 - protein, 17 aa, synthetic construct
  REGION 1..17: note = Description of Artificial Sequence: Synthetic peptide
KSSQSVLFSSNNKNYLA

SEQ ID NO: 347 - protein, 7 aa, synthetic construct
  REGION 1..7: note = Description of Artificial Sequence: Synthetic peptide
WASTRES

SEQ ID NO: 348 - protein, 9 aa, synthetic construct
  REGION 1..9: note = Description of Artificial Sequence: Synthetic peptide
QQFHSYPLT

SEQ ID NO: 349 - protein, 5 aa, synthetic construct
  REGION 1..5: note = Description of Artificial Sequence: Synthetic peptide
SYGMH

SEQ ID NO: 350 - protein, 17 aa, synthetic construct
  REGION 1..17: note = Description of Artificial Sequence: Synthetic peptide
VITYDGINKYYADSVEG

SEQ ID NO: 351 - protein, 10 aa, synthetic construct
  REGION 1..10: note = Description of Artificial Sequence: Synthetic peptide
DGVYYGVYDY

SEQ ID NO: 352 - protein, 17 aa, synthetic construct
  REGION 1..17: note = Description of Artificial Sequence: Synthetic peptide
KSSQSVLFSSNNKNYLA

SEQ ID NO: 353 - protein, 7 aa, synthetic construct
  REGION 1..7: note = Description of Artificial Sequence: Synthetic peptide
WASTRES

SEQ ID NO: 354 - protein, 9 aa, synthetic construct
  REGION 1..9: note = Description of Artificial Sequence: Synthetic peptide
QQFHSYPLT

SEQ ID NO: 355 - protein, 7 aa, synthetic construct
  REGION 1..7: note = Description of Artificial Sequence: Synthetic peptide
GFTFRSY

SEQ ID NO: 356 - protein, 4 aa, synthetic construct
  REGION 1..4: note = Description of Artificial Sequence: Synthetic peptide
YDGI

SEQ ID NO: 357 - protein, 8 aa, synthetic construct
  REGION 1..8: note = Description of Artificial Sequence: Synthetic peptide
GVYYGVYD

SEQ ID NO: 358 - protein, 13 aa, synthetic construct
  REGION 1..13: note = Description of Artificial Sequence: Synthetic peptide
SQSVLFSSNNKNY

SEQ ID NO: 359 - skipped

SEQ ID NO: 360 - protein, 6 aa, synthetic construct
  REGION 1..6: note = Description of Artificial Sequence: Synthetic peptide
FHSYPL

SEQ ID NO: 361 - protein, 10 aa, synthetic construct
  REGION 1..10: note = Description of Artificial Sequence: Synthetic peptide
GFTFRSYGMH

SEQ ID NO: 362 - protein, 10 aa, synthetic construct
  REGION 1..10: note = Description of Artificial Sequence: Synthetic peptide
VITYDGINKY

SEQ ID NO: 363 - protein, 10 aa, synthetic construct
  REGION 1..10: note = Description of Artificial Sequence: Synthetic peptide
DGVYYGVYDY

SEQ ID NO: 364 - protein, 17 aa, synthetic construct
  REGION 1..17: note = Description of Artificial Sequence: Synthetic peptide
KSSQSVLFSSNNKNYLA

SEQ ID NO: 365 - protein, 7 aa, synthetic construct
  REGION 1..7: note = Description of Artificial Sequence: Synthetic peptide
WASTRES

SEQ ID NO: 366 - protein, 9 aa, synthetic construct
  REGION 1..9: note = Description of Artificial Sequence: Synthetic peptide
QQFHSYPLT

SEQ ID NO: 367 - protein, 6 aa, synthetic construct
  REGION 1..6: note = Description of Artificial Sequence: Synthetic peptide
RSYGMH

SEQ ID NO: 368 - protein, 13 aa, synthetic construct
  REGION 1..13: note = Description of Artificial Sequence: Synthetic peptide
WVAVITYDGINKY

SEQ ID NO: 369 - protein, 11 aa, synthetic construct
  REGION 1..11: note = Description of Artificial Sequence: Synthetic peptide
ARDGVYYGVYD

SEQ ID NO: 370 - protein, 13 aa, synthetic construct
  REGION 1..13: note = Description of Artificial Sequence: Synthetic peptide
LFSSNNKNYLAWY

SEQ ID NO: 371 - protein, 10 aa, synthetic construct
  REGION 1..10: note = Description of Artificial Sequence: Synthetic peptide
LLIYWASTRE

SEQ ID NO: 372 - protein, 8 aa, synthetic construct
  REGION 1..8: note = Description of Artificial Sequence: Synthetic peptide
QQFHSYPL

SEQ ID NO: 373 - protein, 8 aa, synthetic construct
  REGION 1..8: note = Description of Artificial Sequence: Synthetic peptide
GFTFRSYG

SEQ ID NO: 374 - protein, 8 aa, synthetic construct
  REGION 1..8: note = Description of Artificial Sequence: Synthetic peptide
ITYDGINK

SEQ ID NO: 375 - protein, 12 aa, synthetic construct
  REGION 1..12: note = Description of Artificial Sequence: Synthetic peptide
ARDGVYYGVYDY

SEQ ID NO: 376 - protein, 12 aa, synthetic construct
  REGION 1..12: note = Description of Artificial Sequence: Synthetic peptide
QSVLFSSNNKNY

SEQ ID NO: 377 - skipped

SEQ ID NO: 378 - protein, 9 aa, synthetic construct
  REGION 1..9: note = Description of Artificial Sequence: Synthetic peptide
QQFHSYPLT

SEQ ID NO: 379 - protein, 119 aa, synthetic construct
  REGION 1..119: note = Description of Artificial Sequence: Synthetic polypeptide
QVQLVESGGGVVQPGRSLRLSCAASGFTFRSYGMHWVRQAPGKGLEWVAVITYDGINKYYADSVEGRFTISRDNSKNTLYLQMNSLRAEDTAVYYCARDGVYYGVYDYWGQGTLVTVSS

SEQ ID NO: 380 - protein, 113 aa, synthetic construct; identical to SEQ ID NO: 342
  REGION 1..113: note = Description of Artificial Sequence: Synthetic polypeptide

SEQ ID NO: 381 - protein, 10 aa, synthetic construct
  REGION 1..10: note = Description of Artificial Sequence: Synthetic peptide
GGTFSSNAIG

SEQ ID NO: 382 - protein, 17 aa, synthetic construct
  REGION 1..17: note = Description of Artificial Sequence: Synthetic peptide
SIIPIIGFANYAQKFQG

SEQ ID NO: 383 - protein, 15 aa, synthetic construct
  REGION 1..15: note = Description of Artificial Sequence: Synthetic peptide
DSGYYYGASSFGMDV

SEQ ID NO: 384 - protein, 11 aa, synthetic construct
  REGION 1..11: note = Description of Artificial Sequence: Synthetic peptide
RASQSVSSNLA

SEQ ID NO: 385 - protein, 7 aa, synthetic construct
  REGION 1..7: note = Description of Artificial Sequence: Synthetic peptide
GASTRAT

SEQ ID NO: 386 - protein, 9 aa, synthetic construct
  REGION 1..9: note = Description of Artificial Sequence: Synthetic peptide
EQYNNLPLT

SEQ ID NO: 387 - protein, 5 aa, synthetic construct
  REGION 1..5: note = Description of Artificial Sequence: Synthetic peptide
SNAIG

SEQ ID NO: 388 - protein, 17 aa, synthetic construct
  REGION 1..17: note = Description of Artificial Sequence: Synthetic peptide
SIIPIIGFANYAQKFQG

SEQ ID NO: 389 - protein, 15 aa, synthetic construct
  REGION 1..15: note = Description of Artificial Sequence: Synthetic peptide
DSGYYYGASSFGMDV

SEQ ID NO: 390 - protein, 11 aa, synthetic construct
  REGION 1..11: note = Description of Artificial Sequence: Synthetic peptide
RASQSVSSNLA

SEQ ID NO: 391 - protein, 7 aa, synthetic construct
  REGION 1..7: note = Description of Artificial Sequence: Synthetic peptide
GASTRAT

SEQ ID NO: 392 - protein, 9 aa, synthetic construct
  REGION 1..9: note = Description of Artificial Sequence: Synthetic peptide
EQYNNLPLT

SEQ ID NO: 393 - protein, 7 aa, synthetic construct
  REGION 1..7: note = Description of Artificial Sequence: Synthetic peptide
GGTFSSN

SEQ ID NO: 394 - protein, 4 aa, synthetic construct
  REGION 1..4: note = Description of Artificial Sequence: Synthetic peptide
PIIG

SEQ ID NO: 395 - protein, 13 aa, synthetic construct
  REGION 1..13: note = Description of Artificial Sequence: Synthetic peptide
SGYYYGASSFGMD

SEQ ID NO: 396 - protein, 7 aa, synthetic construct
  REGION 1..7: note = Description of Artificial Sequence: Synthetic peptide
SQSVSSN

SEQ ID NO: 397 - skipped

SEQ ID NO: 398 - protein, 6 aa, synthetic construct
  REGION 1..6: note = Description of Artificial Sequence: Synthetic peptide
YNNLPL

SEQ ID NO: 399 - protein, 10 aa, synthetic construct
  REGION 1..10: note = Description of Artificial Sequence: Synthetic peptide
GGTFSSNAIG

SEQ ID NO: 400 - protein, 10 aa, synthetic construct
  REGION 1..10: note = Description of Artificial Sequence: Synthetic peptide
SIIPIIGFAN

SEQ ID NO: 401 - protein, 15 aa, synthetic construct
  REGION 1..15: note = Description of Artificial Sequence: Synthetic peptide
DSGYYYGASSFGMDV

SEQ ID NO: 402 - protein, 11 aa, synthetic construct
  REGION 1..11: note = Description of Artificial Sequence: Synthetic peptide
RASQSVSSNLA

SEQ ID NO: 403 - protein, 7 aa, synthetic construct
  REGION 1..7: note = Description of Artificial Sequence: Synthetic peptide
GASTRAT

SEQ ID NO: 404 - protein, 9 aa, synthetic construct
  REGION 1..9: note = Description of Artificial Sequence: Synthetic peptide
EQYNNLPLT

SEQ ID NO: 405 - protein, 6 aa, synthetic construct
  REGION 1..6: note = Description of Artificial Sequence: Synthetic peptide
SSNAIG

SEQ ID NO: 406 - protein, 13 aa, synthetic construct
  REGION 1..13: note = Description of Artificial Sequence: Synthetic peptide
WMGSIIPIIGFAN

SEQ ID NO: 407 - protein, 16 aa, synthetic construct
  REGION 1..16: note = Description of Artificial Sequence: Synthetic peptide
ARDSGYYYGASSFGMD

SEQ ID NO: 408 - protein, 7 aa, synthetic construct
  REGION 1..7: note = Description of Artificial Sequence: Synthetic peptide
SSNLAWY

SEQ ID NO: 409 - protein, 10 aa, synthetic construct
  REGION 1..10: note = Description of Artificial Sequence: Synthetic peptide
LLIYGASTRA

SEQ ID NO: 410 - protein, 8 aa, synthetic construct
  REGION 1..8: note = Description of Artificial Sequence: Synthetic peptide
EQYNNLPL

SEQ ID NO: 411 - protein, 8 aa, synthetic construct
  REGION 1..8: note = Description of Artificial Sequence: Synthetic peptide
GGTFSSNA

SEQ ID NO: 412 - protein, 8 aa, synthetic construct
  REGION 1..8: note = Description of Artificial Sequence: Synthetic peptide
IIPIIGFA

SEQ ID NO: 413 - protein, 17 aa, synthetic construct
  REGION 1..17: note = Description of Artificial Sequence: Synthetic peptide
ARDSGYYYGASSFGMDV

SEQ ID NO: 414 - protein, 6 aa, synthetic construct
  REGION 1..6: note = Description of Artificial Sequence: Synthetic peptide
QSVSSN

SEQ ID NO: 415 - skipped

SEQ ID NO: 416 - protein, 9 aa, synthetic construct
  REGION 1..9: note = Description of Artificial Sequence: Synthetic peptide
EQYNNLPLT

SEQ ID NO: 417 - protein, 124 aa, synthetic construct
  REGION 1..124: note = Description of Artificial Sequence: Synthetic polypeptide
QVQLVQSGAEVKKPGSSVKVSCKASGGTFSSNAIGWVRQAPGQGLEWMGSIIPIIGFANYAQKFQGRVTITADESTSTAYMELSSLRSEDTAVYYCARDSGYYYGASSFGMDVWGQGTTVTVSS

SEQ ID NO: 418 - protein, 107 aa, synthetic construct
  REGION 1..107: note = Description of Artificial Sequence: Synthetic polypeptide
EIVMTQSPATLSVSPGERATLSCRASQSVSSNLAWYQQKPGQAPRLLIYGASTRATGIPARFSGSGSGTEFTLTISSLQSEDFAVYYCEQYNNLPLTFGGGTKVEIK

SEQ ID NO: 419 - protein, 11 aa, synthetic construct
  REGION 1..11: note = Description of Artificial Sequence: Synthetic peptide
GGSISSGQYWS

SEQ ID NO: 420 - protein, 16 aa, synthetic construct
  REGION 1..16: note = Description of Artificial Sequence: Synthetic peptide
EIYYSGSTRYNPSLKS

SEQ ID NO: 421 - protein, 16 aa, synthetic construct
  REGION 1..16: note = Description of Artificial Sequence: Synthetic peptide
DAPYYYGGGYYYYMDV

SEQ ID NO: 422 - protein, 12 aa, synthetic construct
  REGION 1..12: note = Description of Artificial Sequence: Synthetic peptide
RASQSVSSSYLA

SEQ ID NO: 423 - protein, 7 aa, synthetic construct
  REGION 1..7: note = Description of Artificial Sequence: Synthetic peptide
GASSRAT

SEQ ID NO: 424 - protein, 9 aa, synthetic construct
  REGION 1..9: note = Description of Artificial Sequence: Synthetic peptide
QQVGVVPYT

SEQ ID NO: 425 - protein, 6 aa, synthetic construct
  REGION 1..6: note = Description of Artificial Sequence: Synthetic peptide
SGQYWS

SEQ ID NO: 426 - protein, 16 aa, synthetic construct
  REGION 1..16: note = Description of Artificial Sequence: Synthetic peptide
EIYYSGSTRYNPSLKS

SEQ ID NO: 427 - protein, 16 aa, synthetic construct
  REGION 1..16: note = Description of Artificial Sequence: Synthetic peptide
DAPYYYGGGYYYYMDV

SEQ ID NO: 428 - protein, 12 aa, synthetic construct
  REGION 1..12: note = Description of Artificial Sequence: Synthetic peptide
RASQSVSSSYLA

SEQ ID NO: 429 - protein, 7 aa, synthetic construct
  REGION 1..7: note = Description of Artificial Sequence: Synthetic peptide
GASSRAT

SEQ ID NO: 430 - protein, 9 aa, synthetic construct
  REGION 1..9: note = Description of Artificial Sequence: Synthetic peptide
QQVGVVPYT

SEQ ID NO: 431 - protein, 8 aa, synthetic construct
  REGION 1..8: note = Description of Artificial Sequence: Synthetic peptide
GGSISSGQ

SEQ ID NO: 432 - skipped

SEQ ID NO: 433 - protein, 14 aa, synthetic construct
  REGION 1..14: note = Description of Artificial Sequence: Synthetic peptide
APYYYGGGYYYYMD

SEQ ID NO: 434 - protein, 8 aa, synthetic construct
  REGION 1..8: note = Description of Artificial Sequence: Synthetic peptide
SQSVSSSY

SEQ ID NO: 435 - skipped

SEQ ID NO: 436 - protein, 6 aa, synthetic construct
  REGION 1..6: note = Description of Artificial Sequence: Synthetic peptide
VGVVPY

SEQ ID NO: 437 - protein, 11 aa, synthetic construct
  REGION 1..11: note = Description of Artificial Sequence: Synthetic peptide
GGSISSGQYWS

SEQ ID NO: 438 - protein, 9 aa, synthetic construct
  REGION 1..9: note = Description of Artificial Sequence: Synthetic peptide
EIYYSGSTR

SEQ ID NO: 439 - protein, 16 aa, synthetic construct
  REGION 1..16: note = Description of Artificial Sequence: Synthetic peptide
DAPYYYGGGYYYYMDV

SEQ ID NO: 440 - protein, 12 aa, synthetic construct
  REGION 1..12: note = Description of Artificial Sequence: Synthetic peptide
RASQSVSSSYLA

SEQ ID NO: 441 - protein, 7 aa, synthetic construct
  REGION 1..7: note = Description of Artificial Sequence: Synthetic peptide
GASSRAT

SEQ ID NO: 442 - protein, 9 aa, synthetic construct
  REGION 1..9: note = Description of Artificial Sequence: Synthetic peptide
QQVGVVPYT

SEQ ID NO: 443 - protein, 7 aa, synthetic construct
  REGION 1..7: note = Description of Artificial Sequence: Synthetic peptide
SSGQYWS

SEQ ID NO: 444 - protein, 12 aa, synthetic construct
  REGION 1..12: note = Description of Artificial Sequence: Synthetic peptide
WIGEIYYSGSTR

SEQ ID NO: 445 - protein, 17 aa, synthetic construct
  REGION 1..17: note = Description of Artificial Sequence: Synthetic peptide
ARDAPYYYGGGYYYYMD

SEQ ID NO: 446 - protein, 8 aa, synthetic construct
  REGION 1..8: note = Description of Artificial Sequence: Synthetic peptide
SSSYLAWY

SEQ ID NO: 447 - protein, 10 aa, synthetic construct
  REGION 1..10: note = Description of Artificial Sequence: Synthetic peptide
LLIYGASSRA

SEQ ID NO: 448 - protein, 8 aa, synthetic construct
  REGION 1..8: note = Description of Artificial Sequence: Synthetic peptide
QQVGVVPY

SEQ ID NO: 449 - protein, 9 aa, synthetic construct
  REGION 1..9: note = Description of Artificial Sequence: Synthetic peptide
GGSISSGQY

SEQ ID NO: 450 - protein, 7 aa, synthetic construct
  REGION 1..7: note = Description of Artificial Sequence: Synthetic peptide
IYYSGST

SEQ ID NO: 451 - protein, 18 aa, synthetic construct
  REGION 1..18: note = Description of Artificial Sequence: Synthetic peptide
ARDAPYYYGGGYYYYMDV

SEQ ID NO: 452 - protein, 7 aa, synthetic construct
  REGION 1..7: note = Description of Artificial Sequence: Synthetic peptide
QSVSSSY

SEQ ID NO: 453 - skipped

SEQ ID NO: 454 - protein, 9 aa, synthetic construct
  REGION 1..9: note = Description of Artificial Sequence: Synthetic peptide
QQVGVVPYT

SEQ ID NO: 455 - protein, 125 aa, synthetic construct
  REGION 1..125: note = Description of Artificial Sequence: Synthetic polypeptide
QVQLQESGPGLVKPSQTLSLTCTVSGGSISSGQYWSWIRQHPGKGLEWIGEIYYSGSTRYNPSLKSRVTISVDTSKNQFSLKLSSVTAADTAVYYCARDAPYYYGGGYYYYMDVWGKGTTVTVSS

SEQ ID NO: 456 - protein, 108 aa, synthetic construct
  REGION 1..108: note = Description of Artificial Sequence: Synthetic polypeptide
EIVLTQSPGTLSLSPGERATLSCRASQSVSSSYLAWYQQKPGQAPRLLIYGASSRATGIPDRFSGSGSGTDFTLTISRLEPEDFAVYYCQQVGVVPYTFGGGTKVEIK

SEQ ID NO: 457 - protein, 11 aa, synthetic construct
  REGION 1..11: note = Description of Artificial Sequence: Synthetic peptide
GGSISSGQYWS

SEQ ID NO: 458 - protein, 16 aa, synthetic construct
  REGION 1..16: note = Description of Artificial Sequence: Synthetic peptide
EIYYSGSTRYNPSLKS

SEQ ID NO: 459 - protein, 16 aa, synthetic construct
  REGION 1..16: note = Description of Artificial Sequence: Synthetic peptide
DAPYYYGGGYYYYMDV

SEQ ID NO: 460 - protein, 12 aa, synthetic construct
  REGION 1..12: note = Description of Artificial Sequence: Synthetic peptide
RASESVDSSYLA

SEQ ID NO: 461 - protein, 7 aa, synthetic construct
  REGION 1..7: note = Description of Artificial Sequence: Synthetic peptide
GASTRQT

SEQ ID NO: 462 - protein, 9 aa, synthetic construct
  REGION 1..9: note = Description of Artificial Sequence: Synthetic peptide
QQAGVVPYT

SEQ ID NO: 463 - protein, 6 aa, synthetic construct
  REGION 1..6: note = Description of Artificial Sequence: Synthetic peptide
SGQYWS

SEQ ID NO: 464 - protein, 16 aa, synthetic construct
  REGION 1..16: note = Description of Artificial Sequence: Synthetic peptide
EIYYSGSTRYNPSLKS

SEQ ID NO: 465 - protein, 16 aa, synthetic construct
  REGION 1..16: note = Description of Artificial Sequence: Synthetic peptide
DAPYYYGGGYYYYMDV

SEQ ID NO: 466 - protein, 12 aa, synthetic construct
  REGION 1..12: note = Description of Artificial Sequence: Synthetic peptide
RASESVDSSYLA

SEQ ID NO: 467 - protein, 7 aa, synthetic construct
  REGION 1..7: note = Description of Artificial Sequence: Synthetic peptide
GASTRQT

SEQ ID NO: 468 - protein, 9 aa, synthetic construct
  REGION 1..9: note = Description of Artificial Sequence: Synthetic peptide
QQAGVVPYT

SEQ ID NO: 469 - protein, 8 aa, synthetic construct
  REGION 1..8: note = Description of Artificial Sequence: Synthetic peptide
GGSISSGQ

SEQ ID NO: 470 - skipped

SEQ ID NO: 471 - protein, 14 aa, synthetic construct
  REGION 1..14: note = Description of Artificial Sequence: Synthetic peptide
APYYYGGGYYYYMD

SEQ ID NO: 472 - protein, 8 aa, synthetic construct
  REGION 1..8: note = Description of Artificial Sequence: Synthetic peptide
SESVDSSY

SEQ ID NO: 473 - skipped

SEQ ID NO: 474 - protein, 6 aa, synthetic construct
  REGION 1..6: note = Description of Artificial Sequence: Synthetic peptide
AGVVPY

SEQ ID NO: 475 - protein, 11 aa, synthetic construct
  REGION 1..11: note = Description of Artificial Sequence: Synthetic peptide
GGSISSGQYWS

SEQ ID NO: 476 - protein, 9 aa, synthetic construct
  REGION 1..9: note = Description of Artificial Sequence: Synthetic peptide
EIYYSGSTR

SEQ ID NO: 477 - protein, 16 aa, synthetic construct
  REGION 1..16: note = Description of Artificial Sequence: Synthetic peptide
DAPYYYGGGYYYYMDV

SEQ ID NO: 478 - protein, 12 aa, synthetic construct
  REGION 1..12: note = Description of Artificial Sequence: Synthetic peptide
RASESVDSSYLA

SEQ ID NO: 479 - protein, 7 aa, synthetic construct
  REGION 1..7: note = Description of Artificial Sequence: Synthetic peptide
GASTRQT

SEQ ID NO: 480 - protein, 9 aa, synthetic construct
  REGION 1..9: note = Description of Artificial Sequence: Synthetic peptide
QQAGVVPYT

SEQ ID NO: 481 - protein, 7 aa, synthetic construct
  REGION 1..7: note = Description of Artificial Sequence: Synthetic peptide
SSGQYWS

SEQ ID NO: 482 - protein, 12 aa, synthetic construct
  REGION 1..12: note = Description of Artificial Sequence: Synthetic peptide
WIGEIYYSGSTR

SEQ ID NO: 483 - protein, 17 aa, synthetic construct
  REGION 1..17: note = Description of Artificial Sequence: Synthetic peptide
ARDAPYYYGGGYYYYMD

SEQ ID NO: 484 - protein, 8 aa, synthetic construct
  REGION 1..8: note = Description of Artificial Sequence: Synthetic peptide
DSSYLAWY

SEQ ID NO: 485 - protein, 10 aa, synthetic construct
  REGION 1..10: note = Description of Artificial Sequence: Synthetic peptide
LLIYGASTRQ

SEQ ID NO: 486 - protein, 8 aa, synthetic construct
  REGION 1..8: note = Description of Artificial Sequence: Synthetic peptide
QQAGVVPY

SEQ ID NO: 487 - protein, 9 aa, synthetic construct
  REGION 1..9: note = Description of Artificial Sequence: Synthetic peptide
GGSISSGQY

SEQ ID NO: 488 - protein, 7 aa, synthetic construct
  REGION 1..7: note = Description of Artificial Sequence: Synthetic peptide
IYYSGST

SEQ ID NO: 489 - protein, 18 aa, synthetic construct
  REGION 1..18: note = Description of Artificial Sequence: Synthetic peptide
ARDAPYYYGGGYYYYMDV

SEQ ID NO: 490 - protein, 7 aa, synthetic construct
  REGION 1..7: note = Description of Artificial Sequence: Synthetic peptide
ESVDSSY

SEQ ID NO: 491 - skipped

SEQ ID NO: 492 - protein, 9 aa, synthetic construct
  REGION 1..9: note = Description of Artificial Sequence: Synthetic peptide
QQAGVVPYT

SEQ ID NO: 493 - protein, 125 aa, synthetic construct; identical to SEQ ID NO: 455
  REGION 1..125: note = Description of Artificial Sequence: Synthetic polypeptide

SEQ ID NO: 494 - protein, 108 aa, synthetic construct
  REGION 1..108: note = Description of Artificial Sequence: Synthetic polypeptide
EIVLTQSPGTLSLSPGERATLSCRASESVDSSYLAWYQQKPGQAPRLLIYGASTRQTGIPDRFSGSGSGTDFTLTISRLEPEDFAVYYCQQAGVVPYTFGGGTKVEIK

SEQ ID NO: 495 - protein, 11 aa, synthetic construct
  REGION 1..11: note = Description of Artificial Sequence: Synthetic peptide
GGSISSGQYWS

SEQ ID NO: 496 - protein, 16 aa, synthetic construct
  REGION 1..16: note = Description of Artificial Sequence: Synthetic peptide
EIYYSGSTRYNPSLKS

SEQ ID NO: 497 - protein, 16 aa, synthetic construct
  REGION 1..16: note = Description of Artificial Sequence: Synthetic peptide
DAPYYYGGGYYYYMDV

SEQ ID NO: 498 - protein, 12 aa, synthetic construct
  REGION 1..12: note = Description of Artificial Sequence: Synthetic peptide
RASESVDSSYLA

SEQ ID NO: 499 - protein, 7 aa, synthetic construct
  REGION 1..7: note = Description of Artificial Sequence: Synthetic peptide
GADSRAT

SEQ ID NO: 500 - protein, 9 aa, synthetic construct
  REGION 1..9: note = Description of Artificial Sequence: Synthetic peptide
QQDGVVPYT

SEQ ID NO: 501 - protein, 6 aa, synthetic construct
  REGION 1..6: note = Description of Artificial Sequence: Synthetic peptide
SGQYWS

SEQ ID NO: 502 - protein, 16 aa, synthetic construct
  REGION 1..16: note = Description of Artificial Sequence: Synthetic peptide
EIYYSGSTRYNPSLKS

SEQ ID NO: 503 - protein, 16 aa, synthetic construct
  REGION 1..16: note = Description of Artificial Sequence: Synthetic peptide
DAPYYYGGGYYYYMDV

SEQ ID NO: 504 - protein, 12 aa, synthetic construct
  REGION 1..12: note = Description of Artificial Sequence: Synthetic peptide
RASESVDSSYLA

SEQ ID NO: 505 - protein, 7 aa, synthetic construct
  REGION 1..7: note = Description of Artificial Sequence: Synthetic peptide
GADSRAT

SEQ ID NO: 506 - protein, 9 aa, synthetic construct
  REGION 1..9: note = Description of Artificial Sequence: Synthetic peptide
QQDGVVPYT

SEQ ID NO: 507 - protein, 8 aa, synthetic construct
  REGION 1..8: note = Description of Artificial Sequence: Synthetic peptide
GGSISSGQ

SEQ ID NO: 508 - skipped

SEQ ID NO: 509 - protein, 14 aa, synthetic construct
  REGION 1..14: note = Description of Artificial Sequence: Synthetic peptide
APYYYGGGYYYYMD

SEQ ID NO: 510 - protein, 8 aa, synthetic construct
  REGION 1..8: note = Description of Artificial Sequence: Synthetic peptide
SESVDSSY

SEQ ID NO: 511 - skipped

SEQ ID NO: 512 - protein, 6 aa, synthetic construct
  REGION 1..6: note = Description of Artificial Sequence: Synthetic peptide
DGVVPY

SEQ ID NO: 513 - protein, 11 aa, synthetic construct
  REGION 1..11: note = Description of Artificial Sequence: Synthetic peptide
GGSISSGQYWS

SEQ ID NO: 514 - protein, 9 aa, synthetic construct
  REGION 1..9: note = Description of Artificial Sequence: Synthetic peptide
EIYYSGSTR

SEQ ID NO: 515 - protein, 16 aa, synthetic construct
  REGION 1..16: note = Description of Artificial Sequence: Synthetic peptide
DAPYYYGGGYYYYMDV

SEQ ID NO: 516 - protein, 12 aa, synthetic construct
  REGION 1..12: note = Description of Artificial Sequence: Synthetic peptide
RASESVDSSYLA

SEQ ID NO: 517 - protein, 7 aa, synthetic construct
  REGION 1..7: note = Description of Artificial Sequence: Synthetic peptide
GADSRAT

SEQ ID NO: 518 - protein, 9 aa, synthetic construct
  REGION 1..9: note = Description of Artificial Sequence: Synthetic peptide
QQDGVVPYT

SEQ ID NO: 519 - protein, 7 aa, synthetic construct
  REGION 1..7: note = Description of Artificial Sequence: Synthetic peptide
SSGQYWS

SEQ ID NO: 520 - protein, 12 aa, synthetic construct
  REGION 1..12: note = Description of Artificial Sequence: Synthetic peptide
WIGEIYYSGSTR

SEQ ID NO: 521 - protein, 17 aa, synthetic construct
  REGION 1..17: note = Description of Artificial Sequence: Synthetic peptide
ARDAPYYYGGGYYYYMD

SEQ ID NO: 522 - protein, 8 aa, synthetic construct
  REGION 1..8: note = Description of Artificial Sequence: Synthetic peptide
DSSYLAWY

SEQ ID NO: 523 - protein, 10 aa, synthetic construct
  REGION 1..10: note = Description of Artificial Sequence: Synthetic peptide
LLIYGADSRA

SEQ ID NO: 524 - protein, 8 aa, synthetic construct
  REGION 1..8: note = Description of Artificial Sequence: Synthetic peptide
QQDGVVPY

SEQ ID NO: 525 - protein, 9 aa, synthetic construct
  REGION 1..9: note = Description of Artificial Sequence: Synthetic peptide
GGSISSGQY

SEQ ID NO: 526 - protein, 7 aa, synthetic construct
  REGION 1..7: note = Description of Artificial Sequence: Synthetic peptide
IYYSGST

SEQ ID NO: 527 - protein, 18 aa, synthetic construct
  REGION 1..18: note = Description of Artificial Sequence: Synthetic peptide
ARDAPYYYGGGYYYYMDV

SEQ ID NO: 528 - protein, 7 aa, synthetic construct
  REGION 1..7: note = Description of Artificial Sequence: Synthetic peptide
ESVDSSY

SEQ ID NO: 529 - skipped

SEQ ID NO: 530 - protein, 9 aa, synthetic construct
  REGION 1..9: note = Description of Artificial Sequence: Synthetic peptide
QQDGVVPYT

SEQ ID NO: 531 - protein, 125 aa, synthetic construct; identical to SEQ ID NO: 455
  REGION 1..125: note = Description of Artificial Sequence: Synthetic polypeptide

SEQ ID NO: 532 - protein, 108 aa, synthetic construct
  REGION 1..108: note = Description of Artificial Sequence: Synthetic polypeptide
EIVLTQSPGTLSLSPGERATLSCRASESVDSSYLAWYQQKPGQAPRLLIYGADSRATGIPDRFSGSGSGTDFTLTISRLEPEDFAVYYCQQDGVVPYTFGGGTKVEIK

SEQ ID NO: 533 - protein, 10 aa, synthetic construct
  REGION 1..10: note = Description of Artificial Sequence: Synthetic peptide
GGSLSGYYWS

SEQ ID NO: 534 - protein, 16 aa, synthetic construct
  REGION 1..16: note = Description of Artificial Sequence: Synthetic peptide
EIGASGSTRYNPSLKS

SEQ ID NO: 535 - protein, 16 aa, synthetic construct
  REGION 1..16: note = Description of Artificial Sequence: Synthetic peptide
DTPYYYEGGYYYYMDV

SEQ ID NO: 536 - protein, 12 aa, synthetic construct
  REGION 1..12: note = Description of Artificial Sequence: Synthetic peptide
RASQSVSSSYLA

SEQ ID NO: 537 - protein, 7 aa, synthetic construct
  REGION 1..7: note = Description of Artificial Sequence: Synthetic peptide
GASSRAT

SEQ ID NO: 538 - protein, 9 aa, synthetic construct
  REGION 1..9: note = Description of Artificial Sequence: Synthetic peptide
QQVGVVPYT

SEQ ID NO: 539 - protein, 5 aa, synthetic construct
  REGION 1..5: note = Description of Artificial Sequence: Synthetic peptide
GYYWS

SEQ ID NO: 540 - protein, 16 aa, synthetic construct
  REGION 1..16: note = Description of Artificial Sequence: Synthetic peptide
EIGASGSTRYNPSLKS

SEQ ID NO: 541 - protein, 16 aa, synthetic construct
  REGION 1..16: note = Description of Artificial Sequence: Synthetic peptide
DTPYYYEGGYYYYMDV

SEQ ID NO: 542 - protein, 12 aa, synthetic construct
  REGION 1..12: note = Description of Artificial Sequence: Synthetic peptide
RASQSVSSSYLA

SEQ ID NO: 543 - protein, 7 aa, synthetic construct
  REGION 1..7: note = Description of Artificial Sequence: Synthetic peptide
GASSRAT

SEQ ID NO: 544 - protein, 9 aa, synthetic construct
  REGION 1..9: note = Description of Artificial Sequence: Synthetic peptide
QQVGVVPYT

SEQ ID NO: 545 - protein, 7 aa, synthetic construct
  REGION 1..7: note = Description of Artificial Sequence: Synthetic peptide
GGSLSGY

SEQ ID NO: 546 - skipped

SEQ ID NO: 547 - protein, 14 aa, synthetic construct
  REGION 1..14: note = Description of Artificial Sequence: Synthetic peptide
TPYYYEGGYYYYMD

SEQ ID NO: 548 - protein, 8 aa, synthetic construct
  REGION 1..8: note = Description of Artificial Sequence: Synthetic peptide
SQSVSSSY

SEQ ID NO: 549 - skipped

SEQ ID NO: 550 - protein, 6 aa, synthetic construct
  REGION 1..6: note = Description of Artificial Sequence: Synthetic peptide
VGVVPY

SEQ ID NO: 551 - protein, 10 aa, synthetic construct
  REGION 1..10: note = Description of Artificial Sequence: Synthetic peptide
GGSLSGYYWS

SEQ ID NO: 552 - protein, 9 aa, synthetic construct
  REGION 1..9: note = Description of Artificial Sequence: Synthetic peptide
EIGASGSTR

SEQ ID NO: 553 - protein, 16 aa, synthetic construct
  REGION 1..16: note = Description of Artificial Sequence: Synthetic peptide
DTPYYYEGGYYYYMDV

SEQ ID NO: 554 - protein, 12 aa, synthetic construct
  REGION 1..12: note = Description of Artificial Sequence: Synthetic peptide
RASQSVSSSYLA

SEQ ID NO: 555 - protein, 7 aa, synthetic construct
  REGION 1..7: note = Description of Artificial Sequence: Synthetic peptide
GASSRAT

SEQ ID NO: 556 - protein, 9 aa, synthetic construct
  REGION 1..9: note = Description of Artificial Sequence: Synthetic peptide
QQVGVVPYT

SEQ ID NO: 557 - protein, 6 aa, synthetic construct
  REGION 1..6: note = Description of Artificial Sequence: Synthetic peptide
SGYYWS

SEQ ID NO: 558 - protein, 12 aa, synthetic construct
  REGION 1..12: note = Description of Artificial Sequence: Synthetic peptide
WIGEIGASGSTR

SEQ ID NO: 559 - protein, 17 aa, synthetic construct
  REGION 1..17: note = Description of Artificial Sequence: Synthetic peptide
ARDTPYYYEGGYYYYMD

SEQ ID NO: 560 - protein, 8 aa, synthetic construct
  REGION 1..8: note = Description of Artificial Sequence: Synthetic peptide
SSSYLAWY

SEQ ID NO: 561 - protein, 10 aa, synthetic construct
  REGION 1..10: note = Description of Artificial Sequence: Synthetic peptide
LLIYGASSRA

SEQ ID NO: 562 - protein, 8 aa, synthetic construct
  REGION 1..8: note = Description of Artificial Sequence: Synthetic peptide
QQVGVVPY

SEQ ID NO: 563 - protein, 8 aa, synthetic construct
  REGION 1..8: note = Description of Artificial Sequence: Synthetic peptide
GGSLSGYY

SEQ ID NO: 564 - protein, 7 aa, synthetic construct
  REGION 1..7: note = Description of Artificial Sequence: Synthetic peptide
IGASGST

SEQ ID NO: 565 - protein, 18 aa, synthetic construct
  REGION 1..18: note = Description of Artificial Sequence: Synthetic peptide
ARDTPYYYEGGYYYYMDV

SEQ ID NO: 566 - protein, 7 aa, synthetic construct
  REGION 1..7: note = Description of Artificial Sequence: Synthetic peptide
QSVSSSY

SEQ ID NO: 567 - skipped

SEQ ID NO: 568 - protein, 9 aa, synthetic construct
  REGION 1..9: note = Description of Artificial Sequence: Synthetic peptide
QQVGVVPYT

SEQ ID NO: 569 - protein, 124 aa, synthetic construct
  REGION 1..124: note = Description of Artificial Sequence: Synthetic polypeptide
QVQLQQWGAGLLKPSETLSLTCAVYGGSLSGYYWSWIRQPPGKGLEWIGEIGASGSTRYNPSLKSRVTISVDTSKNQFSLKLSSVTAADTAVYYCARDTPYYYEGGYYYYMDVWGKGTTVTVSS

SEQ ID NO: 570 - protein, 108 aa, synthetic construct; identical to SEQ ID NO: 456
  REGION 1..108: note = Description of Artificial Sequence: Synthetic polypeptide

SEQ ID NO: 571 - protein, 10 aa, synthetic construct
  REGION 1..10: note = Description of Artificial Sequence: Synthetic peptide
GGSLSGYYWS

SEQ ID NO: 572 - protein, 16 aa, synthetic construct
  REGION 1..16: note = Description of Artificial Sequence: Synthetic peptide
EIGASGSTRYNPSLKS

SEQ ID NO: 573 - protein, 16 aa, synthetic construct
  REGION 1..16: note = Description of Artificial Sequence: Synthetic peptide
DTPYYYEGGYYYYMDV

SEQ ID NO: 574 - protein, 12 aa, synthetic construct
  REGION 1..12: note = Description of Artificial Sequence: Synthetic peptide
RASDSVDSSYLA

SEQ ID NO: 575 - protein, 7 aa, synthetic construct
  REGION 1..7: note = Description of Artificial Sequence: Synthetic peptide
GAFSRAN

SEQ ID NO: 576 - protein, 9 aa, synthetic construct
  REGION 1..9: note = Description of Artificial Sequence: Synthetic peptide
QQAGVVPYT

SEQ ID NO: 577 - protein, 5 aa, synthetic construct
  REGION 1..5: note = Description of Artificial Sequence: Synthetic peptide
GYYWS

SEQ ID NO: 578 - protein, 16 aa, synthetic construct
  REGION 1..16: note = Description of Artificial Sequence: Synthetic peptide
EIGASGSTRYNPSLKS

SEQ ID NO: 579 - protein, 16 aa, synthetic construct
  REGION 1..16: note = Description of Artificial Sequence: Synthetic peptide
DTPYYYEGGYYYYMDV

SEQ ID NO: 580 - protein, 12 aa, synthetic construct
  REGION 1..12: note = Description of Artificial Sequence: Synthetic peptide
RASDSVDSSYLA

SEQ ID NO: 581 - protein, 7 aa, synthetic construct
  REGION 1..7: note = Description of Artificial Sequence: Synthetic peptide
GAFSRAN

SEQ ID NO: 582 - protein, 9 aa, synthetic construct
  REGION 1..9: note = Description of Artificial Sequence: Synthetic peptide
QQAGVVPYT

SEQ ID NO: 583 - protein, 7 aa, synthetic construct
  REGION 1..7: note = Description of Artificial Sequence: Synthetic peptide
GGSLSGY

SEQ ID NO: 584 - skipped

SEQ ID NO: 585 - protein, 14 aa, synthetic construct
  REGION 1..14: note = Description of Artificial Sequence: Synthetic peptide
TPYYYEGGYYYYMD

SEQ ID NO: 586 - protein, 8 aa, synthetic construct
  REGION 1..8: note = Description of Artificial Sequence: Synthetic peptide
SDSVDSSY

SEQ ID NO: 587 - skipped

SEQ ID NO: 588 - protein, 6 aa, synthetic construct
  REGION 1..6: note = Description of Artificial Sequence: Synthetic peptide
AGVVPY

SEQ ID NO: 589 - protein, 10 aa, synthetic construct
  REGION 1..10: note = Description of Artificial Sequence: Synthetic peptide
GGSLSGYYWS

SEQ ID NO: 590 - protein, 9 aa, synthetic construct
  REGION 1..9: note = Description of Artificial Sequence: Synthetic peptide
EIGASGSTR

SEQ ID NO: 591 - protein, 16 aa, synthetic construct
  REGION 1..16: note = Description of Artificial Sequence: Synthetic peptide
DTPYYYEGGYYYYMDV

SEQ ID NO: 592 - protein, 12 aa, synthetic construct
  REGION 1..12: note = Description of Artificial Sequence: Synthetic peptide
RASDSVDSSYLA

SEQ ID NO: 593 - protein, 7 aa, synthetic construct
  REGION 1..7: note = Description of Artificial Sequence: Synthetic peptide
GAFSRAN

SEQ ID NO: 594 - protein, 9 aa, synthetic construct
  REGION 1..9: note = Description of Artificial Sequence: Synthetic peptide
QQAGVVPYT

SEQ ID NO: 595 - protein, 6 aa, synthetic construct
  REGION 1..6: note = Description of Artificial Sequence: Synthetic peptide
SGYYWS

SEQ ID NO: 596 - protein, 12 aa, synthetic construct
  REGION 1..12: note = Description of Artificial Sequence: Synthetic peptide
WIGEIGASGSTR

SEQ ID NO: 597 - protein, 17 aa, synthetic construct
  REGION 1..17: note = Description of Artificial Sequence: Synthetic peptide
ARDTPYYYEGGYYYYMD

SEQ ID NO: 598 - protein, 8 aa, synthetic construct
  REGION 1..8: note = Description of Artificial Sequence: Synthetic peptide
DSSYLAWY

SEQ ID NO: 599 - protein, 10 aa, synthetic construct
  REGION 1..10: note = Description of Artificial Sequence: Synthetic peptide
LLIYGAFSRA

SEQ ID NO: 600 - protein, 8 aa, synthetic construct
  REGION 1..8: note = Description of Artificial Sequence: Synthetic peptide
QQAGVVPY

SEQ ID NO: 601 - protein, 8 aa, synthetic construct
  REGION 1..8: note = Description of Artificial Sequence: Synthetic peptide
GGSLSGYY

SEQ ID NO: 602 - protein, 7 aa, synthetic construct
  REGION 1..7: note = Description of Artificial Sequence: Synthetic peptide
IGASGST

SEQ ID NO: 603 - protein, 18 aa, synthetic construct
  REGION 1..18: note = Description of Artificial Sequence: Synthetic peptide
ARDTPYYYEGGYYYYMDV

SEQ ID NO: 604 - protein, 7 aa, synthetic construct
  REGION 1..7: note = Description of Artificial Sequence: Synthetic peptide
DSVDSSY

SEQ ID NO: 605 - skipped

SEQ ID NO: 606 - protein, 9 aa, synthetic construct
  REGION 1..9: note = Description of Artificial Sequence: Synthetic peptide
QQAGVVPYT

SEQ ID NO: 607 - protein, 124 aa, synthetic construct; identical to SEQ ID NO: 569
  REGION 1..124: note = Description of Artificial Sequence: Synthetic polypeptide

SEQ ID NO: 608 - protein, 108 aa, synthetic construct
  REGION 1..108: note = Description of Artificial Sequence: Synthetic polypeptide
EIVLTQSPGTLSLSPGERATLSCRASDSVDSSYLAWYQQKPGQAPRLLIYGAFSRANGIPDRFSGSGSGTDFTLTISRLEPEDFAVYYCQQAGVVPYTFGGGTKVEIK

SEQ ID NO: 609 - protein, 10 aa, synthetic construct
  REGION 1..10: note = Description of Artificial Sequence: Synthetic peptide
GGSLSGYYWS

SEQ ID NO: 610 - protein, 16 aa, synthetic construct
  REGION 1..16: note = Description of Artificial Sequence: Synthetic peptide
EIGASGSTRYNPSLKS

SEQ ID NO: 611 - protein, 16 aa, synthetic construct
  REGION 1..16: note = Description of Artificial Sequence: Synthetic peptide
DTPYYYEGGYYYYMDV

SEQ ID NO: 612 - protein, 12 aa, synthetic construct
  REGION 1..12: note = Description of Artificial Sequence: Synthetic peptide
RASQSVSSSFLA

SEQ ID NO: 613 - protein, 7 aa, synthetic construct
  REGION 1..7: note = Description of Artificial Sequence: Synthetic peptide
GAYSRAT

SEQ ID NO: 614 - protein, 9 aa, synthetic construct
  REGION 1..9: note = Description of Artificial Sequence: Synthetic peptide
QQAGVVPYT

SEQ ID NO: 615 - protein, 5 aa, synthetic construct
  REGION 1..5: note = Description of Artificial Sequence: Synthetic peptide
GYYWS

SEQ ID NO: 616 - protein, 16 aa, synthetic construct
  REGION 1..16: note = Description of Artificial Sequence: Synthetic peptide
EIGASGSTRYNPSLKS

SEQ ID NO: 617 - protein, 16 aa, synthetic construct
  REGION 1..16: note = Description of Artificial Sequence: Synthetic peptide
DTPYYYEGGYYYYMDV

SEQ ID NO: 618 - protein, 12 aa, synthetic construct
  REGION 1..12: note = Description of Artificial Sequence: Synthetic peptide
RASQSVSSSFLA

SEQ ID NO: 619 - protein, 7 aa, synthetic construct
  REGION 1..7: note = Description of Artificial Sequence: Synthetic peptide
GAYSRAT

SEQ ID NO: 620 - protein, 9 aa, synthetic construct
  REGION 1..9: note = Description of Artificial Sequence: Synthetic peptide
QQAGVVPYT

SEQ ID NO: 621 - protein, 7 aa, synthetic construct
  REGION 1..7: note = Description of Artificial Sequence: Synthetic peptide
GGSLSGY

SEQ ID NO: 622 - skipped

SEQ ID NO: 623 - protein, 14 aa, synthetic construct
  REGION 1..14: note = Description of Artificial Sequence: Synthetic peptide
TPYYYEGGYYYYMD

SEQ ID NO: 624 - protein, 8 aa, synthetic construct
  REGION 1..8: note = Description of Artificial Sequence: Synthetic peptide
SQSVSSSF

SEQ ID NO: 625 - skipped

SEQ ID NO: 626 - protein, 6 aa, synthetic construct
  REGION 1..6: note = Description of Artificial Sequence: Synthetic peptide
AGVVPY

SEQ ID NO: 627 - protein, 10 aa, synthetic construct
  REGION 1..10: note = Description of Artificial Sequence: Synthetic peptide
GGSLSGYYWS

SEQ ID NO: 628 - protein, 9 aa, synthetic construct
  REGION 1..9: note = Description of Artificial Sequence: Synthetic peptide
EIGASGSTR

SEQ ID NO: 629 - protein, 16 aa, synthetic construct
  REGION 1..16: note = Description of Artificial Sequence: Synthetic peptide
DTPYYYEGGYYYYMDV

SEQ ID NO: 630 - protein, 12 aa, synthetic construct
  REGION 1..12: note = Description of Artificial Sequence: Synthetic peptide
RASQSVSSSFLA

SEQ ID NO: 631 - protein, 7 aa, synthetic construct
  REGION 1..7: note = Description of Artificial Sequence: Synthetic peptide
GAYSRAT

SEQ ID NO: 632 - protein, 9 aa, synthetic construct
  REGION 1..9: note = Description of Artificial Sequence: Synthetic peptide
QQAGVVPYT

SEQ ID NO: 633 - protein, 6 aa, synthetic construct
  REGION 1..6: note = Description of Artificial Sequence: Synthetic peptide
SGYYWS

SEQ ID NO: 634 - protein, 12 aa, synthetic construct
  REGION 1..12: note = Description of Artificial Sequence: Synthetic peptide
WIGEIGASGSTR

SEQ ID NO: 635 - protein, 17 aa, synthetic construct
  REGION 1..17: note = Description of Artificial Sequence: Synthetic peptide
ARDTPYYYEGGYYYYMD

SEQ ID NO: 636 - protein, 8 aa, synthetic construct
  REGION 1..8: note = Description of Artificial Sequence: Synthetic peptide
SSSFLAWY

SEQ ID NO: 637 - protein, 10 aa, synthetic construct
  REGION 1..10: note = Description of Artificial Sequence: Synthetic peptide
LLIYGAYSRA

SEQ ID NO: 638 - protein, 8 aa, synthetic construct
  REGION 1..8: note = Description of Artificial Sequence: Synthetic peptide
QQAGVVPY

SEQ ID NO: 639 - protein, 8 aa, synthetic construct
  REGION 1..8: note = Description of Artificial Sequence: Synthetic peptide
GGSLSGYY

SEQ ID NO: 640 - protein, 7 aa, synthetic construct
  REGION 1..7: note = Description of Artificial Sequence: Synthetic peptide
IGASGST

SEQ ID NO: 641 - protein, 18 aa, synthetic construct
  REGION 1..18: note = Description of Artificial Sequence: Synthetic peptide
ARDTPYYYEGGYYYYMDV

SEQ ID NO: 642 - protein, 7 aa, synthetic construct
  REGION 1..7: note = Description of Artificial Sequence: Synthetic peptide
QSVSSSF

SEQ ID NO: 643 - skipped

SEQ ID NO: 644 - protein, 9 aa, synthetic construct
  REGION 1..9: note = Description of Artificial Sequence: Synthetic peptide
QQAGVVPYT

SEQ ID NO: 645 - protein, 124 aa, synthetic construct; identical to SEQ ID NO: 569
  REGION 1..124: note = Description of Artificial Sequence: Synthetic polypeptide

SEQ ID NO: 646 - protein, 108 aa, synthetic construct
  REGION 1..108: note = Description of Artificial Sequence: Synthetic polypeptide
EIVLTQSPGTLSLSPGERATLSCRASQSVSSSFLAWYQQKPGQAPRLLIYGAYSRATGIPDRFSGSGSGTDFTLTISRLEPEDFAVYYCQQAGVVPYTFGGGTKVEIK

SEQ ID NO: 647 - protein, 11 aa, synthetic construct
  REGION 1..11: note = Description of Artificial Sequence: Synthetic peptide
GGSISSGQYWS

SEQ ID NO: 648 - protein, 16 aa, synthetic construct
  REGION 1..16: note = Description of Artificial Sequence: Synthetic peptide
EIYYSGSTRYNPSLKS

SEQ ID NO: 649 - protein, 16 aa, synthetic construct
  REGION 1..16: note = Description of Artificial Sequence: Synthetic peptide
DTPYYYDGGYYYYMDV

SEQ ID NO: 650 - protein, 12 aa, synthetic construct
  REGION 1..12: note = Description of Artificial Sequence: Synthetic peptide
RASQSVSSSYLA

SEQ ID NO: 651 - protein, 7 aa, synthetic construct
  REGION 1..7: note = Description of Artificial Sequence: Synthetic peptide
GASSRAT

SEQ ID NO: 652 - protein, 9 aa, synthetic construct
  REGION 1..9: note = Description of Artificial Sequence: Synthetic peptide
QQVGVVPYT

SEQ ID NO: 653 - protein, 6 aa, synthetic construct
  REGION 1..6: note = Description of Artificial Sequence: Synthetic peptide
SGQYWS

SEQ ID NO: 654 - protein, 16 aa, synthetic construct
  REGION 1..16: note = Description of Artificial Sequence: Synthetic peptide
EIYYSGSTRYNPSLKS

SEQ ID NO: 655 - protein, 16 aa, synthetic construct
  REGION 1..16: note = Description of Artificial Sequence: Synthetic peptide
DTPYYYDGGYYYYMDV

SEQ ID NO: 656 - protein, 12 aa, synthetic construct
  REGION 1..12: note = Description of Artificial Sequence: Synthetic peptide
RASQSVSSSYLA

SEQ ID NO: 657 - protein, 7 aa, synthetic construct
  REGION 1..7: note = Description of Artificial Sequence: Synthetic peptide
GASSRAT

SEQ ID NO: 658 - protein, 9 aa, synthetic construct
  REGION 1..9: note = Description of Artificial Sequence: Synthetic peptide
QQVGVVPYT

SEQ ID NO: 659 - protein, 8 aa, synthetic construct
  REGION 1..8: note = Description of Artificial Sequence: Synthetic peptide
GGSISSGQ

SEQ ID NO: 660 - skipped

SEQ ID NO: 661 - protein, 14 aa, synthetic construct
  REGION 1..14: note = Description of Artificial Sequence: Synthetic peptide
TPYYYDGGYYYYMD

SEQ ID NO: 662 - protein, 8 aa, synthetic construct
  REGION 1..8: note = Description of Artificial Sequence: Synthetic peptide
SQSVSSSY

SEQ ID NO: 663 - skipped

SEQ ID NO: 664 - protein, 6 aa, synthetic construct
  REGION 1..6: note = Description of Artificial Sequence: Synthetic peptide
VGVVPY

SEQ ID NO: 665 - protein, 11 aa, synthetic construct
  REGION 1..11: note = Description of Artificial Sequence: Synthetic peptide
GGSISSGQYWS

SEQ ID NO: 666 - protein, 9 aa, synthetic construct
  REGION 1..9: note = Description of Artificial Sequence: Synthetic peptide
EIYYSGSTR

SEQ ID NO: 667 - protein, 16 aa, synthetic construct
  REGION 1..16: note = Description of Artificial Sequence: Synthetic peptide
DTPYYYDGGYYYYMDV

SEQ ID NO: 668 - protein, 12 aa, synthetic construct
  REGION 1..12: note = Description of Artificial Sequence: Synthetic peptide
RASQSVSSSYLA

SEQ ID NO: 669 - protein, 7 aa, synthetic construct
  REGION 1..7: note = Description of Artificial Sequence: Synthetic peptide
GASSRAT

SEQ ID NO: 670 - protein, 9 aa, synthetic construct
  REGION 1..9: note = Description of Artificial Sequence: Synthetic peptide
QQVGVVPYT

SEQ ID NO: 671 - protein, 7 aa, synthetic construct
  REGION 1..7: note = Description of Artificial Sequence: Synthetic peptide
SSGQYWS

SEQ ID NO: 672 - protein, 12 aa, synthetic construct
  REGION 1..12: note = Description of Artificial Sequence: Synthetic peptide
WIGEIYYSGSTR

SEQ ID NO: 673 - protein, 17 aa, synthetic construct
  REGION 1..17: note = Description of Artificial Sequence: Synthetic peptide
ARDTPYYYDGGYYYYMD

SEQ ID NO: 674 - protein, 8 aa, synthetic construct
  REGION 1..8: note = Description of Artificial Sequence: Synthetic peptide
SSSYLAWY

SEQ ID NO: 675 - protein, 10 aa, synthetic construct
  REGION 1..10: note = Description of Artificial Sequence: Synthetic peptide
LLIYGASSRA

SEQ ID NO: 676 - protein, 8 aa, synthetic construct
  REGION 1..8: note = Description of Artificial Sequence: Synthetic peptide
QQVGVVPY

SEQ ID NO: 677 - protein, 9 aa, synthetic construct
  REGION 1..9: note = Description of Artificial Sequence: Synthetic peptide
GGSISSGQY

SEQ ID NO: 678 - protein, 7 aa, synthetic construct
  REGION 1..7: note = Description of Artificial Sequence: Synthetic peptide
IYYSGST

SEQ ID NO: 679 - protein, 18 aa, synthetic construct
  REGION 1..18: note = Description of Artificial Sequence: Synthetic peptide
ARDTPYYYDGGYYYYMDV

SEQ ID NO: 680 - protein, 7 aa, synthetic construct
  REGION 1..7: note = Description of Artificial Sequence: Synthetic peptide
QSVSSSY

SEQ ID NO: 681 - skipped

SEQ ID NO: 682 - protein, 9 aa, synthetic construct
  REGION 1..9: note = Description of Artificial Sequence: Synthetic peptide
QQVGVVPYT

SEQ ID NO: 683 - protein, 125 aa, synthetic construct
  REGION 1..125: note = Description of Artificial Sequence: Synthetic polypeptide
QVQLQESGPGLVKPSQTLSLTCTVSGGSISSGQYWSWIRQHPGKGLEWIGEIYYSGSTRYNPSLKSRVTISVDTSKDQFSLKLSSVTAADTAVYYCARDTPYYYDGGYYYYMDVWGKGTTVTVSS

SEQ ID NO: 684 - protein, 108 aa, synthetic construct; identical to SEQ ID NO: 456
  REGION 1..108: note = Description of Artificial Sequence: Synthetic polypeptide

SEQ ID NO: 685 - protein, 11 aa, synthetic construct
  REGION 1..11: note = Description of Artificial Sequence: Synthetic peptide
GGSISSGQYWS

SEQ ID NO: 686 - protein, 16 aa, synthetic construct
  REGION 1..16: note = Description of Artificial Sequence: Synthetic peptide
EIYYSGSTRYNPSLKS

SEQ ID NO: 687 - protein, 16 aa, synthetic construct
  REGION 1..16: note = Description of Artificial Sequence: Synthetic peptide
DTPYYYDGGYYYYMDV

SEQ ID NO: 688 - protein, 12 aa, synthetic construct
  REGION 1..12: note = Description of Artificial Sequence: Synthetic peptide
RASQSVSSSYLA

SEQ ID NO: 689 - protein, 7 aa, synthetic construct
  REGION 1..7: note = Description of Artificial Sequence: Synthetic peptide
GASSRAT

SEQ ID NO: 690 - protein, 9 aa, synthetic construct
  REGION 1..9: note = Description of Artificial Sequence: Synthetic peptide
QQVGVVPYT

SEQ ID NO: 691 - protein, 6 aa, synthetic construct
  REGION 1..6: note = Description of Artificial Sequence: Synthetic peptide
SGQYWS

SEQ ID NO: 692 - protein, 16 aa, synthetic construct
  REGION 1..16: note = Description of Artificial Sequence: Synthetic peptide
EIYYSGSTRYNPSLKS

SEQ ID NO: 693 - protein, 16 aa, synthetic construct
  REGION 1..16: note = Description of Artificial Sequence: Synthetic peptide
DTPYYYDGGYYYYMDV

SEQ ID NO: 694 - protein, 12 aa, synthetic construct
  REGION 1..12: note = Description of Artificial Sequence: Synthetic peptide
RASQSVSSSYLA

SEQ ID NO: 695 - protein, 7 aa, synthetic construct
  REGION 1..7: note = Description of Artificial Sequence: Synthetic peptide
GASSRAT

SEQ ID NO: 696 - protein, 9 aa, synthetic construct
  REGION 1..9: note = Description of Artificial Sequence: Synthetic peptide
QQVGVVPYT

SEQ ID NO: 697 - protein, 8 aa, synthetic construct
  REGION 1..8: note = Description of Artificial Sequence: Synthetic peptide
GGSISSGQ

SEQ ID NO: 698 - skipped

SEQ ID NO: 699 - protein, 14 aa, synthetic construct
  REGION 1..14: note = Description of Artificial Sequence: Synthetic peptide
TPYYYDGGYYYYMD

SEQ ID NO: 700 - protein, 8 aa, synthetic construct
  REGION 1..8: note = Description of Artificial Sequence: Synthetic peptide
SQSVSSSY

SEQ ID NO: 701 - skipped

SEQ ID NO: 702 - protein, 6 aa, synthetic construct
  REGION 1..6: note = Description of Artificial Sequence: Synthetic peptide
VGVVPY

SEQ ID NO: 703 - protein, 11 aa, synthetic construct
  REGION 1..11: note = Description of Artificial Sequence: Synthetic peptide
GGSISSGQYWS

SEQ ID NO: 704 - protein, 9 aa, synthetic construct
  REGION 1..9: note = Description of Artificial Sequence: Synthetic peptide
EIYYSGSTR

SEQ ID NO: 705 - protein, 16 aa, synthetic construct
  REGION 1..16: note = Description of Artificial Sequence: Synthetic peptide
DTPYYYDGGYYYYMDV

SEQ ID NO: 706 - protein, 12 aa, synthetic construct
  REGION 1..12: note = Description of Artificial Sequence: Synthetic peptide
RASQSVSSSYLA

SEQ ID NO: 707 - protein, 7 aa, synthetic construct
  REGION 1..7: note = Description of Artificial Sequence: Synthetic peptide
GASSRAT

SEQ ID NO: 708 - protein, 9 aa, synthetic construct
  REGION 1..9: note = Description of Artificial Sequence: Synthetic peptide
QQVGVVPYT

SEQ ID NO: 709 - protein, 7 aa, synthetic construct
  REGION 1..7: note = Description of Artificial Sequence: Synthetic peptide
SSGQYWS

SEQ ID NO: 710 - protein, 12 aa, synthetic construct
  REGION 1..12: note = Description of Artificial Sequence: Synthetic peptide
WIGEIYYSGSTR

SEQ ID NO: 711 - protein, 17 aa, synthetic construct
  REGION 1..17: note = Description of Artificial Sequence: Synthetic peptide
ARDTPYYYDGGYYYYMD

SEQ ID NO: 712 - protein, 8 aa, synthetic construct
  REGION 1..8: note = Description of Artificial Sequence: Synthetic peptide
SSSYLAWY

SEQ ID NO: 713 - protein, 10 aa, synthetic construct
  REGION 1..10: note = Description of Artificial Sequence: Synthetic peptide
LLIYGASSRA

SEQ ID NO: 714 - protein, 8 aa, synthetic construct
  REGION 1..8: note = Description of Artificial Sequence: Synthetic peptide
QQVGVVPY

SEQ ID NO: 715 - protein, 9 aa, synthetic construct
  REGION 1..9: note = Description of Artificial Sequence: Synthetic peptide
GGSISSGQY

SEQ ID NO: 716 - protein, 7 aa, synthetic construct
  REGION 1..7: note = Description of Artificial Sequence: Synthetic peptide
IYYSGST

SEQ ID NO: 717 - protein, 18 aa, synthetic construct
  REGION 1..18: note = Description of Artificial Sequence: Synthetic peptide
ARDTPYYYDGGYYYYMDV

SEQ ID NO: 718 - protein, 7 aa, synthetic construct
  REGION 1..7: note = Description of Artificial Sequence: Synthetic peptide
QSVSSSY

SEQ ID NO: 719 - skipped

SEQ ID NO: 720 - protein, 9 aa, synthetic construct
  REGION 1..9: note = Description of Artificial Sequence: Synthetic peptide
QQVGVVPYT

SEQ ID NO: 721 - protein, 125 aa, synthetic construct
  REGION 1..125: note = Description of Artificial Sequence: Synthetic polypeptide
QVQLQESGPGLVKPSQTLSLTCTVSGGSISSGQYWSWIRQHPGKGLEWIGEIYYSGSTRYNPSLKSRVTISVDTSKNQFSLKLSSVTAADTAVYYCARDTPYYYDGGYYYYMDVWGKGTTVTVSS

SEQ ID NO: 722 - protein, 108 aa, synthetic construct; identical to SEQ ID NO: 456
  REGION 1..108: note = Description of Artificial Sequence: Synthetic polypeptide

SEQ ID NO: 723 - protein, 10 aa, synthetic construct
  REGION 1..10: note = Description of Artificial Sequence: Synthetic peptide
GYTFANYYMH

SEQ ID NO: 724 - protein, 17 aa, synthetic construct
  REGION 1..17: note = Description of Artificial Sequence: Synthetic peptide
IINPSGGITVYAQKFQG

SEQ ID NO: 725 - protein, 12 aa, synthetic construct
  REGION 1..12: note = Description of Artificial Sequence: Synthetic peptide
GGSKVAALAFDI

SEQ ID NO: 726 - protein, 11 aa, synthetic construct
  REGION 1..11: note = Description of Artificial Sequence: Synthetic peptide
QASQDISNSLN

SEQ ID NO: 727 - protein, 7 aa, synthetic construct
  REGION 1..7: note = Description of Artificial Sequence: Synthetic peptide
DASNLET

SEQ ID NO: 728 - protein, 9 aa, synthetic construct
  REGION 1..9: note = Description of Artificial Sequence: Synthetic peptide
QQYNFHPLT

SEQ ID NO: 729 - protein, 5 aa, synthetic construct
  REGION 1..5: note = Description of Artificial Sequence: Synthetic peptide
NYYMH

SEQ ID NO: 730 - protein, 17 aa, synthetic construct
  REGION 1..17: note = Description of Artificial Sequence: Synthetic peptide
IINPSGGITVYAQKFQG

SEQ ID NO: 731 - protein, 12 aa, synthetic construct
  REGION 1..12: note = Description of Artificial Sequence: Synthetic peptide
GGSKVAALAFDI

SEQ ID NO: 732 - protein, 11 aa, synthetic construct
  REGION 1..11: note = Description of Artificial Sequence: Synthetic peptide
QASQDISNSLN

SEQ ID NO: 733 - protein, 7 aa, synthetic construct
  REGION 1..7: note = Description of Artificial Sequence: Synthetic peptide
DASNLET

SEQ ID NO: 734 - protein, 9 aa, synthetic construct
  REGION 1..9: note = Description of Artificial Sequence: Synthetic peptide
QQYNFHPLT

SEQ ID NO: 735 - protein, 7 aa, synthetic construct
  REGION 1..7: note = Description of Artificial Sequence: Synthetic peptide
GYTFANY

SEQ ID NO: 736 - protein, 4 aa, synthetic construct
  REGION 1..4: note = Description of Artificial Sequence: Synthetic peptide
PSGG

SEQ ID NO: 737 - protein, 10 aa, synthetic construct
  REGION 1..10: note = Description of Artificial Sequence: Synthetic peptide
GSKVAALAFD

SEQ ID NO: 738 - protein, 7 aa, synthetic construct
  REGION 1..7: note = Description of Artificial Sequence: Synthetic peptide
SQDISNS

SEQ ID NO: 739 - skipped

SEQ ID NO: 740 - protein, 6 aa, synthetic construct
  REGION 1..6: note = Description of Artificial Sequence: Synthetic peptide
YNFHPL

SEQ ID NO: 741 - protein, 10 aa, synthetic construct
  REGION 1..10: note = Description of Artificial Sequence: Synthetic peptide
GYTFANYYMH

SEQ ID NO: 742 - protein, 10 aa, synthetic construct
  REGION 1..10: note = Description of Artificial Sequence: Synthetic peptide
IINPSGGITV

SEQ ID NO: 743 - protein, 12 aa, synthetic construct
  REGION 1..12: note = Description of Artificial Sequence: Synthetic peptide
GGSKVAALAFDI

SEQ ID NO: 744 - protein, 11 aa, synthetic construct
  REGION 1..11: note = Description of Artificial Sequence: Synthetic peptide
QASQDISNSLN

SEQ ID NO: 745 - protein, 7 aa, synthetic construct
  REGION 1..7: note = Description of Artificial Sequence: Synthetic peptide
DASNLET

SEQ ID NO: 746 - protein, 9 aa, synthetic construct
  REGION 1..9: note = Description of Artificial Sequence: Synthetic peptide
QQYNFHPLT

SEQ ID NO: 747 - protein, 6 aa, synthetic construct
  REGION 1..6: note = Description of Artificial Sequence: Synthetic peptide
ANYYMH

SEQ ID NO: 748 - protein, 13 aa, synthetic construct
  REGION 1..13: note = Description of Artificial Sequence: Synthetic peptide
WMGIINPSGGITV

SEQ ID NO: 749 - protein, 13 aa, synthetic construct
  REGION 1..13: note = Description of Artificial Sequence: Synthetic peptide
ARGGSKVAALAFD

SEQ ID NO: 750 - protein, 7 aa, synthetic construct
  REGION 1..7: note = Description of Artificial Sequence: Synthetic peptide
SNSLNWY

SEQ ID NO: 751 - protein, 10 aa, synthetic construct
  REGION 1..10: note = Description of Artificial Sequence: Synthetic peptide
LLIYDASNLE

SEQ ID NO: 752 - protein, 8 aa, synthetic construct
  REGION 1..8: note = Description of Artificial Sequence: Synthetic peptide
QQYNFHPL

SEQ ID NO: 753 - protein, 8 aa, synthetic construct
  REGION 1..8: note = Description of Artificial Sequence: Synthetic peptide
GYTFANYY

SEQ ID NO: 754 - protein, 8 aa, synthetic construct
  REGION 1..8: note = Description of Artificial Sequence: Synthetic peptide
INPSGGIT

SEQ ID NO: 755 - protein, 14 aa, synthetic construct
  REGION 1..14: note = Description of Artificial Sequence: Synthetic peptide
ARGGSKVAALAFDI

SEQ ID NO: 756 - protein, 6 aa, synthetic construct
  REGION 1..6: note = Description of Artificial Sequence: Synthetic peptide
QDISNS

SEQ ID NO: 757 - skipped

SEQ ID NO: 758 - protein, 9 aa, synthetic construct
  REGION 1..9: note = Description of Artificial Sequence: Synthetic peptide
QQYNFHPLT

SEQ ID NO: 759 - protein, 121 aa, synthetic construct
  REGION 1..121: note = Description of Artificial Sequence: Synthetic polypeptide
QVQLVQSGAEVKKPGASVKVSCKASGYTFANYYMHWVRQAPGQGLEWMGIINPSGGITVYAQKFQGRVTMTRDTSTSTVYMELSSLRSEDTAVYYCARGGSKVAALAFDIWGQGTMVTVSS

SEQ ID NO: 760 - protein, 107 aa, synthetic construct
  REGION 1..107: note = Description of Artificial Sequence: Synthetic polypeptide
DIQMTQSPSSLSASVGDRVTITCQASQDISNSLNWYQQKPGKAPKLLIYDASNLETGVPSRFSGSRSGTDFTFTISSLQPEDIATYYCQQYNFHPLTFGGGTKVEIK

SEQ ID NO: 761 - protein, 118 aa, synthetic construct
  REGION 1..118: note = Description of Artificial Sequence: Synthetic polypeptide
  MOD_RES 31: note = Asp or Ser
  MOD_RES 35: note = Ala or Gly
  MOD_RES 50: note = Ala or Thr
EVQLLESGGGLVQPGGSLRLSCAASGFTFSXYAMXWVRQAPGKGLEWVSXISGSGGLTYYADSVKGRFTISRDNSKNTLYLQMNSLRAEDTAVYYCAKAPYGYYMDVWGKGTTVTVSS

SEQ ID NO: 762 - protein, 106 aa, synthetic construct; identical to SEQ ID NO: 38
  REGION 1..106: note = Description of Artificial Sequence: Synthetic polypeptide

SEQ ID NO: 763 - protein, 123 aa, synthetic construct
  REGION 1..123: note = Description of Artificial Sequence: Synthetic polypeptide
  MOD_RES 30: note = Asp or Arg
  MOD_RES 31: note = Ser, Val, or Ala
  MOD_RES 51: note = Ile or Val
  MOD_RES 55: note = Ser or Asn
  MOD_RES 106: note = Phe or Tyr
QVQLVQSGAEVKKPGASVKVSCKASGYTFXXYGISWVRQAPGQGLEWMGWXAPYXGNTNYAQKLQGRVTMTTDTSTSTAYMELRSLRSDDTAVYYCARDAGTYSPXGYGMDVWGQGTTVTVSS

SEQ ID NO: 764 - protein, 108 aa, synthetic construct
  REGION 1..108: note = Description of Artificial Sequence: Synthetic polypeptide
  MOD_RES 24: note = Arg or Gln
  MOD_RES 27: note = Gln, Glu, or His
  MOD_RES 30: note = Ser, Asp, or Asn
  MOD_RES 31: note = Ser or Asn
  MOD_RES 50: note = Lys or Ser
  MOD_RES 52: note = Ser or Tyr
  MOD_RES 53: note = Ser, Tyr, or Asn
  MOD_RES 56: note = Ser or Tyr
  MOD_RES 90: note = Gln, Leu, or Arg
  MOD_RES 93: note = Ser or Lys
DIQMTQSPSTLSASVGDRVTITCXASXSIXXWLAWYQQKPGKAPKLLIYXAXXLEXGVPSRFSGSGSGTEFTLTISSLQPDDFATYYCQXFQXLPPFTFGGGTKVEIK

SEQ ID NO: 765 - protein, 119 aa, synthetic construct
  REGION 1..119: note = Description of Artificial Sequence: Synthetic polypeptide
  MOD_RES 30: note = His or Arg
  MOD_RES 32: note = Arg or Tyr
QVQLVESGGGVVQPGRSLRLSCAASGFTFXSXGMHWVRQAPGKGLEWVAVITYDGINKYYADSVEGRFTISRDNSKNTLYLQMNSLRAEDTAVYYCARDGVYYGVYDYWGQGTLVTVSS

SEQ ID NO: 766 - protein, 113 aa, synthetic construct; identical to SEQ ID NO: 342
  REGION 1..113: note = Description of Artificial Sequence: Synthetic polypeptide

SEQ ID NO: 767 - protein, 124 aa, synthetic construct; identical to SEQ ID NO: 417
  REGION 1..124: note = Description of Artificial Sequence: Synthetic polypeptide

SEQ ID NO: 768 - protein, 107 aa, synthetic construct; identical to SEQ ID NO: 418
  REGION 1..107: note = Description of Artificial Sequence: Synthetic polypeptide

SEQ ID NO: 769 - protein, 125 aa, synthetic construct
  REGION 1..125: note = Description of Artificial Sequence: Synthetic polypeptide
  MOD_RES 6: note = Glu or Gln
  MOD_RES 7: note = Ser or Trp
  MOD_RES 9: note = Pro or Ala
  MOD_RES 12: note = Val or Leu
  MOD_RES 16: note = Gln or Glu
  MOD_RES 23: note = Thr or Ala
  MOD_RES 25: note = Ser or Tyr
  MOD_RES 29: note = Ile or Leu
  MOD_RES 33: note = Gln or Tyr
  MOD_RES 41: note = His or Pro
  MOD_RES 53: note = Tyr or Gly
  MOD_RES 54: note = Tyr or Ala
  MOD_RES 77: note = Asn or Asp
  MOD_RES 100: note = Thr or Ala
  MOD_RES 105: note = Glu, Gly, or Asp
QVQLQXXGXGLXKPSXTLSLTCXVXGGSXSSGXYWSWIRQXPGKGLEWIGEIXXSGSTRYNPSLKSRVTISVDTSKXQFSLKLSSVTAADTAVYYCARDXPYYYXGGYYYYMDVWGKGTTVTVSS

SEQ ID NO: 770 - protein, 108 aa, synthetic construct
  REGION 1..108: note = Description of Artificial Sequence: Synthetic polypeptide
  MOD_RES 27: note = Gln, Glu, or Asp
  MOD_RES 30: note = Ser or Asp
  MOD_RES 33: note = Tyr or Phe
  MOD_RES 53: note = Ser, Asp, Phe, or Tyr
  MOD_RES 54: note = Ser or Thr
  MOD_RES 56: note = Ala or Gln
  MOD_RES 57: note = Thr or Asn
  MOD_RES 92: note = Val, Ala, or Asp
EIVLTQSPGTLSLSPGERATLSCRASXSVXSSXLAWYQQKPGQAPRLLIYGAXXRXXGIPDRFSGSGSGTDFTLTISRLEPEDFAVYYCQQXGVVPYTFGGGTKVEIK

SEQ ID NO: 771 - protein, 121 aa, synthetic construct; identical to SEQ ID NO: 759
  REGION 1..121: note = Description of Artificial Sequence: Synthetic polypeptide

SEQ ID NO: 772 - protein, 107 aa, synthetic construct; identical to SEQ ID NO: 760
  REGION 1..107: note = Description of Artificial Sequence: Synthetic polypeptide

SEQ ID NO: 773 - protein, 10 aa, synthetic construct
  REGION 1..10: note = Description of Artificial Sequence: Synthetic peptide
  MOD_RES 6: note = Asp or Ser
  MOD_RES 10: note = Ala or Gly
GFTFSXYAMX

SEQ ID NO: 774 - protein, 17 aa, synthetic construct
  REGION 1..17: note = Description of Artificial Sequence: Synthetic peptide
  MOD_RES 1: note = Ala or Thr
XISGSGGLTYYADSVKG

SEQ ID NO: 775 - protein, 9 aa, synthetic construct
  REGION 1..9: note = Description of Artificial Sequence: Synthetic peptide
APYGYYMDV

SEQ ID NO: 776 - protein, 11 aa, synthetic construct
  REGION 1..11: note = Description of Artificial Sequence: Synthetic peptide
RASQSISSWLA

SEQ ID NO: 777 - protein, 7 aa, synthetic construct
  REGION 1..7: note = Description of Artificial Sequence: Synthetic peptide
KASSLES

SEQ ID NO: 778 - protein, 8 aa, synthetic construct
  REGION 1..8: note = Description of Artificial Sequence: Synthetic peptide
QQYKSYIT

SEQ ID NO: 779 - protein, 10 aa, synthetic construct
  REGION 1..10: note = Description of Artificial Sequence: Synthetic peptide
  MOD_RES 5: note = Asp or Arg
  MOD_RES 6: note = Ser or Val
GYTFXXYGIS

SEQ ID NO: 780 - protein, 17 aa, synthetic construct
  REGION 1..17: note = Description of Artificial Sequence: Synthetic peptide
  MOD_RES 2: note = Ile or Val
  MOD_RES 6: note = Ser or Asn
WXAPYXGNTNYAQKLQG

SEQ ID NO: 781 - protein, 14 aa, synthetic construct
  REGION 1..14: note = Description of Artificial Sequence: Synthetic peptide
  MOD_RES 8: note = Phe or Tyr
DAGTYSPXGYGMDV

SEQ ID NO: 782 - protein, 11 aa, synthetic construct
  REGION 1..11: note = Description of Artificial Sequence: Synthetic peptide
  MOD_RES 1: note = Arg or Gln
  MOD_RES 4: note = Gln, Glu, or His
  MOD_RES 7: note = Ser, Asp, or Asn
  MOD_RES 8: note = Ser or Asn
XASXSIXXWLA

SEQ ID NO: 783 - skipped

SEQ ID NO: 784 - protein, 10 aa, synthetic construct
  REGION 1..10: note = Description of Artificial Sequence: Synthetic peptide
  MOD_RES 2: note = Gln, Leu, or Arg
  MOD_RES 5: note = Ser or Lys
QXFQXLPPFT

SEQ ID NO: 785 - protein, 10 aa, synthetic construct
  REGION 1..10: note = Description of Artificial Sequence: Synthetic peptide
  MOD_RES 5: note = His or Arg
  MOD_RES 7: note = Arg or Tyr
GFTFXSXGMH

SEQ ID NO: 786 - protein, 17 aa, synthetic construct
  REGION 1..17: note = Description of Artificial Sequence: Synthetic peptide
VITYDGINKYYADSVEG

SEQ ID NO: 787 - protein, 10 aa, synthetic construct
  REGION 1..10: note = Description of Artificial Sequence: Synthetic peptide
DGVYYGVYDY

SEQ ID NO: 788 - protein, 17 aa, synthetic construct
  REGION 1..17: note = Description of Artificial Sequence: Synthetic peptide
KSSQSVLFSSNNKNYLA

SEQ ID NO: 789 - protein, 7 aa, synthetic construct
  REGION 1..7: note = Description of Artificial Sequence: Synthetic peptide
WASTRES

SEQ ID NO: 790 - protein, 9 aa, synthetic construct
  REGION 1..9: note = Description of Artificial Sequence: Synthetic peptide
QQFHSYPLT

SEQ ID NO: 791 - protein, 10 aa, synthetic construct
  REGION 1..10: note = Description of Artificial Sequence: Synthetic peptide
GGTFSSNAIG

SEQ ID NO: 792 - protein, 17 aa, synthetic construct
  REGION 1..17: note = Description of Artificial Sequence: Synthetic peptide
SIIPIIGFANYAQKFQG

SEQ ID NO: 793 - protein, 15 aa, synthetic construct
  REGION 1..15: note = Description of Artificial Sequence: Synthetic peptide
DSGYYYGASSFGMDV

SEQ ID NO: 794 - protein, 11 aa, synthetic construct
  REGION 1..11: note = Description of Artificial Sequence: Synthetic peptide
RASQSVSSNLA

SEQ ID NO: 795 - protein, 7 aa, synthetic construct
  REGION 1..7: note = Description of Artificial Sequence: Synthetic peptide
GASTRAT

SEQ ID NO: 796 - protein, 9 aa, synthetic construct
  REGION 1..9: note = Description of Artificial Sequence: Synthetic peptide
EQYNNLPLT

SEQ ID NO: 797 - protein, 11 aa, synthetic construct
  REGION 1..11: note = Description of Artificial Sequence: Synthetic peptide
  MOD_RES 4: note = Ile or Leu
  MOD_RES 8: note = Gln or Tyr
GGSXSSGXYWS

SEQ ID NO: 798 - protein, 16 aa, synthetic construct
  REGION 1..16: note = Description of Artificial Sequence: Synthetic peptide
  MOD_RES 3: note = Tyr or Gly
  MOD_RES 4: note = Tyr or Ala
EIXXSGSTRYNPSLKS

SEQ ID NO: 799 - protein, 16 aa, synthetic construct
  REGION 1..16: note = Description of Artificial Sequence: Synthetic peptide
  MOD_RES 2: note = Thr or Ala
  MOD_RES 7: note = Glu, Gly, or Asp
DXPYYYXGGYYYYMDV

SEQ ID NO: 800 - protein, 12 aa, synthetic construct
  REGION 1..12: note = Description of Artificial Sequence: Synthetic peptide
  MOD_RES 4: note = Gln, Glu, or Asp
  MOD_RES 7: note = Ser or Asp
  MOD_RES 10: note = Tyr or Phe
RASXSVXSSXLA

SEQ ID NO: 801 - skipped

SEQ ID NO: 802 - protein, 9 aa, synthetic construct
  REGION 1..9: note = Description of Artificial Sequence: Synthetic peptide
  MOD_RES 3: note = Val, Ala, or Asp
QQXGVVPYT

SEQ ID NO: 803 - protein, 10 aa, synthetic construct
  REGION 1..10: note = Description of Artificial Sequence: Synthetic peptide
GYTFANYYMH

SEQ ID NO: 804 - protein, 17 aa, synthetic construct
  REGION 1..17: note = Description of Artificial Sequence: Synthetic peptide
IINPSGGITVYAQKFQG

SEQ ID NO: 805 - protein, 12 aa, synthetic construct
  REGION 1..12: note = Description of Artificial Sequence: Synthetic peptide
GGSKVAALAFDI

SEQ ID NO: 806 - protein, 11 aa, synthetic construct
  REGION 1..11: note = Description of Artificial Sequence: Synthetic peptide
QASQDISNSLN

SEQ ID NO: 807 - protein, 7 aa, synthetic construct
  REGION 1..7: note = Description of Artificial Sequence: Synthetic peptide
DASNLET

SEQ ID NO: 808 - protein, 9 aa, synthetic construct
  REGION 1..9: note = Description of Artificial Sequence: Synthetic peptide
QQYNFHPLT

SEQ ID NO: 809 - protein, 295 aa, Homo sapiens
METPAWPRVPRPETAVARTLLLGWVFAQVAGASGTTNTVAAYNLTWKSTNFKTILEWEPKPVNQVYTVQISTKSGDWKSKCFYTTDTECDLTDEIVKDVKQTYLARVFSYPAGNVESTGSAGEPLYENSPEFTPYLETNLGQPTIQSFEQVGTKVNVTVEDERTLVRRNNTFLSLRDVFGKDLIYTLYYWKSSSSGKKTAKTNTNEFLIDVDKGENYCFSVQAVIPSRTVNRKSTDSPVECMGQEKGEFREIFYIIGAVVFVVIILVIILAISLHKCRKAGVGQSWKENSPLNVS

SEQ ID NO: 810 - protein, 219 aa, Homo sapiens
SGTTNTVAAYNLTWKSTNFKTILEWEPKPVNQVYTVQISTKSGDWKSKCFYTTDTECDLTDEIVKDVKQTYLARVFSYPAGNVESTGSAGEPLYENSPEFTPYLETNLGQPTIQSFEQVGTKVNVTVEDERTLVRRNNTFLSLRDVFGKDLIYTLYYWKSSSSGKKTAKTNTNEFLIDVDKGENYCFSVQAVIPSRTVNRKSTDSPVECMGQEKGEFRE

SEQ ID NO: 811 - protein, 227 aa, synthetic construct
  REGION 1..227: note = Description of Artificial Sequence: Synthetic polypeptide
SGTTNTVAAYNLTWKSTNFKTILEWEPKPVNQVYTVQISTKSGDWKSKCFYTTDTECDLTDEIVKDVKQTYLARVFSYPAGNVESTGSAGEPLYENSPEFTPYLETNLGQPTIQSFEQVGTKVNVTVEDERTLVRRNNTFLSLRDVFGKDLIYTLYYWKSSSSGKKTAKTNTNEFLIDVDKGENYCFSVQAVIPSRTVNRKSTDSPVECMGQEKGEFRETGHHHHHH

SEQ ID NO: 812 - protein, 455 aa, synthetic construct
  REGION 1..455: note = Description of Artificial Sequence: Synthetic polypeptide
SGTTNTVAAYNLTWKSTNFKTILEWEPKPVNQVYTVQISTKSGDWKSKCFYTTDTECDLTDEIVKDVKQTYLARVFSYPAGNVESTGSAGEPLYENSPEFTPYLETNLGQPTIQSFEQVGTKVNVTVEDERTLVRRNNTFLSLRDVFGKDLIYTLYYWKSSSSGKKTAKTNTNEFLIDVDKGENYCFSVQAVIPSRTVNRKSTDSPVECMGQEKGEFRETGENLYFQGDKTHTCPPCPAPELLGGPSVFLFPPKPKDTLMISRTPEVTCVVVDVSHEDPEVKFNWYVDGVEVHNAKTKPREEQYNSTYRVVSVLTVLHQDWLNGKEYKCKVSNKALPAPIEKTISKAKGQPREPQVYTLPPSREEMTKNQVSLTCLVKGFYPSDIAVEWESNGQPENNYKTTPPVLDSDGSFFLYSKLTVDKSRWQQGNVFSCSVMHEALHNHYTQKSLSLSPGK

SEQ ID NO: 813 - protein, 296 aa, Macaca fascicularis
METPAWPRVPRPETAVARTLLLGWVFAQVAGASGTTNTVAAYNLTWKSTNFKTILEWEPKPINQVYTVQISTKSGDWKSKCFYTADTECDLTDEIVKDVKQTYLARVFSYPAGHVESTGSTEEPPYENSPEFTPYLETNLGQPTIQSFEQVGTKVNVTVQDEWTLVRRNDTFLSLRDVFGKDLIYTLYYWKSSSSGKKTAKTNTNEFLIDVDKGENYCFSVQAVIPSRRTANRKSTDSPVECMGHEKGESREIFYIIGAVVFVVIILVIILAISLHKCKKARVGRSWKENSPLNVA

SEQ ID NO: 814 - protein, 220 aa, Macaca fascicularis
SGTTNTVAAYNLTWKSTNFKTILEWEPKPINQVYTVQISTKSGDWKSKCFYTADTECDLTDEIVKDVKQTYLARVFSYPAGHVESTGSTEEPPYENSPEFTPYLETNLGQPTIQSFEQVGTKVNVTVQDEWTLVRRNDTFLSLRDVFGKDLIYTLYYWKSSSSGKKTAKTNTNEFLIDVDKGENYCFSVQAVIPSRRTANRKSTDSPVECMGHEKGESRE

SEQ ID NO: 815 - protein, 228 aa, synthetic construct
  REGION 1..228: note = Description of Artificial Sequence: Synthetic polypeptide
SGTTNTVAAYNLTWKSTNFKTILEWEPKPINQVYTVQISTKSGDWKSKCFYTADTECDLTDEIVKDVKQTYLARVFSYPAGHVESTGSTEEPPYENSPEFTPYLETNLGQPTIQSFEQVGTKVNVTVQDEWTLVRRNDTFLSLRDVFGKDLIYTLYYWKSSSSGKKTAKTNTNEFLIDVDKGENYCFSVQAVIPSRRTANRKSTDSPVECMGHEKGESRETGHHHHHH

SEQ ID NO: 816 - protein, 456 aa, synthetic construct
  REGION 1..456: note = Description of Artificial Sequence: Synthetic polypeptide
SGTTNTVAAYNLTWKSTNFKTILEWEPKPINQVYTVQISTKSGDWKSKCFYTADTECDLTDEIVKDVKQTYLARVFSYPAGHVESTGSTEEPPYENSPEFTPYLETNLGQPTIQSFEQVGTKVNVTVQDEWTLVRRNDTFLSLRDVFGKDLIYTLYYWKSSSSGKKTAKTNTNEFLIDVDKGENYCFSVQAVIPSRRTANRKSTDSPVECMGHEKGESRETGENLYFQGDKTHTCPPCPAPELLGGPSVFLFPPKPKDTLMISRTPEVTCVVVDVSHEDPEVKFNWYVDGVEVHNAKTKPREEQYNSTYRVVSVLTVLHQDWLNGKEYKCKVSNKALPAPIEKTISKAKGQPREPQVYTLPPSREEMTKNQVSLTCLVKGFYPSDIAVEWESNGQPENNYKTTPPVLDSDGSFFLYSKLTVDKSRWQQGNVFSCSVMHEALHNHYTQKSLSLSPGK

SEQ ID NO: 817 - protein, 294 aa, Mus musculus
MAILVRPRLLAALAPTFLGCLLLQVTAGAGIPEKAFNLTWISTDFKTILEWQPKPTNYTYTVQISDRSRNWKNKCFSTTDTECDLTDEIVKDVTWAYEAKVLSVPRRNSVHGDGDQLVIHGEEPPFTNAPKFLPYRDTNLGQPVIQQFEQDGRKLNVVVKDSLTLVRKNGTFLTLRQVFGKDLGYIITYRKGSSTGKKTNITNTNEFSIDVEEGVSYCFFVQAMIFSRKTNQNSPGSSTVCTEQWKSFLGETLIIVGAVVLLATIFIILLSISLCKRRKNRAGQKGKNTPSRLA

SEQ ID NO: 818 - protein, 223 aa, Mus musculus
AGIPEKAFNLTWISTDFKTILEWQPKPTNYTYTVQISDRSRNWKNKCFSTTDTECDLTDEIVKDVTWAYEAKVLSVPRRNSVHGDGDQLVIHGEEPPFTNAPKFLPYRDTNLGQPVIQQFEQDGRKLNVVVKDSLTLVRKNGTFLTLRQVFGKDLGYIITYRKGSSTGKKTNITNTNEFSIDVEEGVSYCFFVQAMIFSRKTNQNSPGSSTVCTEQWKSFLGE

SEQ ID NO: 819 - protein, 231 aa, synthetic construct
  REGION 1..231: note = Description of Artificial Sequence: Synthetic polypeptide
AGIPEKAFNLTWISTDFKTILEWQPKPTNYTYTVQISDRSRNWKNKCFSTTDTECDLTDEIVKDVTWAYEAKVLSVPRRNSVHGDGDQLVIHGEEPPFTNAPKFLPYRDTNLGQPVIQQFEQDGRKLNVVVKDSLTLVRKNGTFLTLRQVFGKDLGYIITYRKGSSTGKKTNITNTNEFSIDVEEGVSYCFFVQAMIFSRKTNQNSPGSSTVCTEQWKSFLGETGHHHHHH

SEQ ID NO: 820 - protein, 459 aa, synthetic construct
  REGION 1..459: note = Description of Artificial Sequence: Synthetic polypeptide
AGIPEKAFNLTWISTDFKTILEWQPKPTNYTYTVQISDRSRNWKNKCFSTTDTECDLTDEIVKDVTWAYEAKVLSVPRRNSVHGDGDQLVIHGEEPPFTNAPKFLPYRDTNLGQPVIQQFEQDGRKLNVVVKDSLTLVRKNGTFLTLRQVFGKDLGYIITYRKGSSTGKKTNITNTNEFSIDVEEGVSYCFFVQAMIFSRKTNQNSPGSSTVCTEQWKSFLGETGENLYFQGDKTHTCPPCPAPELLGGPSVFLFPPKPKDTLMISRTPEVTCVVVDVSHEDPEVKFNWYVDGVEVHNAKTKPREEQYNSTYRVVSVLTVLHQDWLNGKEYKCKVSNKALPAPIEKTISKAKGQPREPQVYTLPPSREEMTKNQVSLTCLVKGFYPSDIAVEWESNGQPENNYKTTPPVLDSDGSFFLYSKLTVDKSRWQQGNVFSCSVMHEALHNHYTQKSLSLSPGK

SEQ ID NO: 821 - protein, 120 aa, synthetic construct
  REGION 1..120: note = Description of Artificial Sequence: Synthetic polypeptide
EVQLVQSGAEVKKPGESLRISCKGSGYTFAPYWIEWVRQMPGKGLEWMGDILPGTGFTTYSPSFQGHVTISADKSISTAYLQWSSLKASDTAMYYCARSGYYGNSGFAYWGQGTLVTVSS

SEQ ID NO: 822 - protein, 113 aa, synthetic construct
  REGION 1..113: note = Description of Artificial Sequence: Synthetic polypeptide
DIVMTQTPLSLPVTPGEPASISCKSSQSLLSSGNQKNYLTWYLQKPGQSPQLLIYWASTRESGVPDRFSGSGSGTDFTLKISRVEAEDVGVYYCQNDYTYPLTFGQGTKLEIK

SEQ ID NO: 823 - protein, 5 aa, synthetic construct
  REGION 1..5: note = Description of Artificial Sequence: Synthetic peptide
GGGGS

SEQ ID NO: 824 - protein, 292 aa, Sus scrofa
MATPTGPPVSCPKAAVARALLLGWVLVQVAGATGTTDVIVAYNLTWKSTNFKTILEWEPKPINYVYTVQISPRLGDWKNKCFHTTDTECDVTDEIMRNVKETYVARVLSYPADTVLTAQEPPFTNSPPFTPYLDTNLGQPVIQSFEQVGTKLNVTVEAARTLVRVNGTFLRLRDVFGKDLNYTLYYWRASSTGKKKATTNTNEFLIDVDKGENYCFSVQAVIPSRRVNQKSPESRIECTSQEKAVSRELFLIVGAVVFAVIVFVLVLSVSLYKCRKERAGPSGKENAPLNVA

SEQ ID NO: 825 - protein, 216 aa, Sus scrofa
TGTTDVIVAYNLTWKSTNFKTILEWEPKPINYVYTVQISPRLGDWKNKCFHTTDTECDVTDEIMRNVKETYVARVLSYPADTVLTAQEPPFTNSPPFTPYLDTNLGQPVIQSFEQVGTKLNVTVEAARTLVRVNGTFLRLRDVFGKDLNYTLYYWRASSTGKKKATTNTNEFLIDVDKGENYCFSVQAVIPSRRVNQKSPESRIECTSQEKAVSRE

SEQ ID NO: 826 - protein, 224 aa, synthetic construct
  REGION 1..224: note = Description of Artificial Sequence: Synthetic polypeptide
TGTTDVIVAYNLTWKSTNFKTILEWEPKPINYVYTVQISPRLGDWKNKCFHTTDTECDVTDEIMRNVKETYVARVLSYPADTVLTAQEPPFTNSPPFTPYLDTNLGQPVIQSFEQVGTKLNVTVEAARTLVRVNGTFLRLRDVFGKDLNYTLYYWRASSTGKKKATTNTNEFLIDVDKGENYCFSVQAVIPSRRVNQKSPESRIECTSQEKAVSRETGHHHHHH

SEQ ID NO: 827 - protein, 452 aa, synthetic construct
  REGION 1..452: note = Description of Artificial Sequence: Synthetic polypeptide
TGTTDVIVAYNLTWKSTNFKTILEWEPKPINYVYTVQISPRLGDWKNKCFHTTDTECDVTDEIMRNVKETYVARVLSYPADTVLTAQEPPFTNSPPFTPYLDTNLGQPVIQSFEQVGTKLNVTVEAARTLVRVNGTFLRLRDVFGKDLNYTLYYWRASSTGKKKATTNTNEFLIDVDKGENYCFSVQAVIPSRRVNQKSPESRIECTSQEKAVSRETGENLYFQGDKTHTCPPCPAPELLGGPSVFLFPPKPKDTLMISRTPEVTCVVVDVSHEDPEVKFNWYVDGVEVHNAKTKPREEQYNSTYRVVSVLTVLHQDWLNGKEYKCKVSNKALPAPIEKTISKAKGQPREPQVYTLPPSREEMTKNQVSLTCLVKGFYPSDIAVEWESNGQPENNYKTTPPVLDSDGSFFLYSKLTVDKSRWQQGNVFSCSVMHEALHNHYTQKSLSLSPGK

SEQ ID NO: 828 - protein, 118 aa, synthetic construct
  REGION 1..118: note = Description of Artificial Sequence: Synthetic polypeptide
EVQLLESGGGLVQPGGSLRLSCAASGFTFSNYAMSWVRQAPGKGLEWVSSISGSGDYTYYTDSVKGRFTISRDNSKNTLYLQMNSLRAEDTAVYYCARSPWGYYLDSWGQGTLVTVSS

SEQ ID NO: 829 - protein, 107 aa, synthetic construct
  REGION 1..107: note = Description of Artificial Sequence: Synthetic polypeptide
DIQMTQSPPSLSASAGDRVTITCRASQGISSRLAWYQQKPEKAPKSLIYAASSLQSGVPSRFSGSGSGTDFTLTISSLQPEDFATYYCQQYNSYPYTFGQGTKLEIK

SEQ ID NO: 830 - protein, 117 aa, synthetic construct
  REGION 1..117: note = Description of Artificial Sequence: Synthetic polypeptide
QVQLVESGGGVVQPGRSLRLSCKASGFNIKDYYMHWVRQAPGKGLEWIGLIDPENGNTIYDPKFQGRFTISADNSKNTLFLQMDSLRPEDTAVYYCARDNSYYFDYWGQGTPVTVSS

SEQ ID NO: 831 - protein, 107 aa, synthetic construct
  REGION 1..107: note = Description of Artificial Sequence: Synthetic polypeptide
DIQMTQSPSSLSASVGDRVTITCKASQDIRKYLNWYQQKPGKAPKLLIYYATSLADGVPSRFSGSGSGTDYTFTISSLQPEDIATYYCLQHGESPYTFGQGTKLEIT

SEQ ID NO: 832 - protein, 292 aa, Oryctolagus cuniculus
MAPPTRLQVPRPGTAVPYTVLLGWLLAQVARAADTTGRAYNLTWKSTNFKTILEWEPKSIDHVYTVQISTRLENWKSKCFLTAETECDLTDEVVKDVGQTYMARVLSYPARNGNTTGFPEEPPFRNSPEFTPYLDTNLGQPTIQSFEQVGTKLNVTVQDARTLVRRNGTFLSLRAVFGKDLNYTLYYWRASSTGKKTATTNTNEFLIDVDKGENYCFSVQAVIPSRKRKQRSPESLTECTSREQGRAREMFFIIGAVVVVALLIIVLSVTVYKCRKARAGPSGKESSPLNIA

SEQ ID NO: 833 - protein, 218 aa, Oryctolagus cuniculus
ADTTGRAYNLTWKSTNFKTILEWEPKSIDHVYTVQISTRLENWKSKCFLTAETECDLTDEVVKDVGQTYMARVLSYPARNGNTTGFPEEPPFRNSPEFTPYLDTNLGQPTIQSFEQVGTKLNVTVQDARTLVRRNGTFLSLRAVFGKDLNYTLYYWRASSTGKKTATTNTNEFLIDVDKGENYCFSVQAVIPSRKRKQRSPESLTECTSREQGRAREM

SEQ ID NO: 834 - protein, 226 aa, synthetic construct
  REGION 1..226: note = Description of Artificial Sequence: Synthetic polypeptide
ADTTGRAYNLTWKSTNFKTILEWEPKSIDHVYTVQISTRLENWKSKCFLTAETECDLTDEVVKDVGQTYMARVLSYPARNGNTTGFPEEPPFRNSPEFTPYLDTNLGQPTIQSFEQVGTKLNVTVQDARTLVRRNGTFLSLRAVFGKDLNYTLYYWRASSTGKKTATTNTNEFLIDVDKGENYCFSVQAVIPSRKRKQRSPESLTECTSREQGRAREMTGHHHHHH

SEQ ID NO: 835 - protein, 452 aa, synthetic construct
  REGION 1..452: note = Description of Artificial Sequence: Synthetic polypeptide
ADTTGRAYNLTWKSTNFKTILEWEPKSIDHVYTVQISTRLENWKSKCFLTAETECDLTDEVVKDVGQTYMARVLSYPARNGNTTGFPEEPPFRNSPEFTPYLDTNLGQPTIQSFEQVGTKLNVTVQDARTLVRRNGTFLSLRAVFGKDLNYTLYYWRASSTGKKTATTNTNEFLIDVDKGENYCFSVQAVIPSRKRKQRSPESLTECTSREQGRAREMENLYFQGDKTHTCPPCPAPELLGGPSVFLFPPKPKDTLMISRTPEVTCVVVDVSHEDPEVKFNWYVDGVEVHNAKTKPREEQYNSTYRVVSVLTVLHQDWLNGKEYKCKVSNKALPAPIEKTISKAKGQPREPQVYTLPPSREEMTKNQVSLTCLVKGFYPSDIAVEWESNGQPENNYKTTPPVLDSDGSFFLYSKLTVDKSRWQQGNVFSCSVMHEALHNHYTQKSLSLSPGK

SEQ ID NO: 836 - protein, 123 aa, synthetic construct
  REGION 1..123: note = Description of Artificial Sequence: Synthetic polypeptide
QVQLVQSGAEVKKPGASVKVSCKASGYTFDAYGISWVRQAPGQGLEWMGWIAPYSGNTNYAQKLQGRVTMTTDTSTSTAYMELRSLRSDDTAVYYCARDAGTYSPFGYGMDVWGQGTTVTVSS

SEQ ID NO: 837 - protein, 108 aa, synthetic construct; identical to SEQ ID NO: 190
  REGION 1..108: note = Description of Artificial Sequence: Synthetic polypeptide

SEQ ID NO: 838 - protein, 224 aa, Rattus sp.
AGTPPGKAFNLTWISTDFKTILEWQPKPTNYTYTVQISDRSRNWKYKCTGTTDTECDLTDEIVKDVNWTYEARVLSVPWRNSTHGKETLFGTHGEEPPFTNARKFLPYRDTKIGQPVIQKYEQGGTKLKVTVKDSFTLVRKNGTFLTLRQVFGNDLGYILTYRKDSSTGRKTNTTHTNEFLIDVEKGVSYCFFAQAVIFSRKTNHKSPESITKCTEQWKSVLGE

SEQ ID NO: 839 - protein, 224 aa, synthetic construct
  REGION 1..224: note = Description of Artificial Sequence: Synthetic polypeptide
AGTPPGKAFNLTWISTDFKTILEWQPKPTNYTYTVQISDRSRNWKYKCTGTTDTECDLTDEIVKDVNWTYEARVLSVPWRNSTHGKETLFGTHGEEPPFTNARKFLPYRDTKLGQPTIQSFEQVGTKVNVTVEDERTLVRRNNTFLSLRDVFGKDLIYTLYYWKSSSSGKKTAKTNTNEFLIDVDKGENYCFSVQAVIPSRTVNRKSTDSPVECMGQEKGEFRE

SEQ ID NO: 840 - protein, 218 aa, synthetic construct
  REGION 1..218: note = Description of Artificial Sequence: Synthetic polypeptide
AGTPPGKAFNLTWISTDFKTILEWQPKPTNYTYTVQISDRSRNWKYKCTGTTDTECDLTDEIVKDVNWTYEARVLSYPAGNVESTGSAGEPLYENSPEFTPYLETNLGQPTIQSFEQVGTKVNVTVEDERTLVRRNNTFLSLRDVFGKDLIYTLYYWKSSSSGKKTAKTNTNEFLIDVDKGENYCFSVQAVIPSRTVNRKSTDSPVECMGQEKGEFRE

SEQ ID NO: 841 - protein, 218 aa, synthetic construct
  REGION 1..218: note = Description of Artificial Sequence: Synthetic polypeptide
AGTPPGKAFNLTWISTDFKTILEWQPKPTNYTYTVQISTKSGDWKSKCFYTTDTECDLTDEIVKDVKQTYLARVFSYPAGNVESTGSAGEPLYENSPEFTPYLETNLGQPTIQSFEQVGTKVNVTVEDERTLVRRNNTFLSLRDVFGKDLIYTLYYWKSSSSGKKTAKTNTNEFLIDVDKGENYCFSVQAVIPSRTVNRKSTDSPVECMGQEKGEFRE

SEQ ID NO: 842 - protein, 219 aa, synthetic construct
  REGION 1..219: note = Description of Artificial Sequence: Synthetic polypeptide
SGTTNTVAAYNLTWKSTNFKTILEWEPKPVNQVYTVQISDRSRNWKYKCTGTTDTECDLTDEIVKDVNWTYEARVLSYPAGNVESTGSAGEPLYENSPEFTPYLETNLGQPTIQSFEQVGTKVNVTVEDERTLVRRNNTFLSLRDVFGKDLIYTLYYWKSSSSGKKTAKTNTNEFLIDVDKGENYCFSVQAVIPSRTVNRKSTDSPVECMGQEKGEFRE

SEQ ID NO: 843 - protein, 219 aa, synthetic construct
  REGION 1..219: note = Description of Artificial Sequence: Synthetic polypeptide
SGTTNTVAAYNLTWKSTNFKTILEWEPKPVNQVYTVQISTKSGDWKSKCFYTTDTECDLTDEIVKDVKQTYLARVFSVPWRNSTHGTHGEEPPFTNARKFLPYRDTKLGQPTIQSFEQVGTKVNVTVEDERTLVRRNNTFLSLRDVFGKDLIYTLYYWKSSSSGKKTAKTNTNEFLIDVDKGENYCFSVQAVIPSRTVNRKSTDSPVECMGQEKGEFRE

SEQ ID NO: 844 - protein, 225 aa, synthetic construct
  REGION 1..225: note = Description of Artificial Sequence: Synthetic polypeptide
SGTTNTVAAYNLTWKSTNFKTILEWEPKPVNQVYTVQISTKSGDWKSKCFYTTDTECDLTDEIVKDVKQTYLARVFSVPWRNSTHGKETLFGTHGEEPPFTNARKFLPYRDTKLGQPTIQSFEQVGTKVNVTVEDERTLVRRNNTFLSLRDVFGKDLIYTLYYWKSSSSGKKTAKTNTNEFLIDVDKGENYCFSVQAVIPSRTVNRKSTDSPVECMGQEKGEFRE

SEQ ID NO: 845 - protein, 225 aa, synthetic construct
  REGION 1..225: note = Description of Artificial Sequence: Synthetic polypeptide
SGTTNTVAAYNLTWKSTNFKTILEWEPKPVNQVYTVQISTKSGDWKSKCFYTTDTECDLTDEIVKDVKQTYLARVFSVPWRNSTHGKETLFGTHGEEPPYENSPEFTPYLETNLGQPTIQSFEQVGTKVNVTVEDERTLVRRNNTFLSLRDVFGKDLIYTLYYWKSSSSGKKTAKTNTNEFLIDVDKGENYCFSVQAVIPSRTVNRKSTDSPVECMGQEKGEFRE

SEQ ID NO: 846 - protein, 219 aa, synthetic construct
  REGION 1..219: note = Description of Artificial Sequence: Synthetic polypeptide
SGTTNTVAAYNLTWKSTNFKTILEWEPKPVNQVYTVQISTKSGDWKSKCFYTTDTECDLTDEIVKDVKQTYLARVFSYPAGNVESTGSAGEPLFTNARKFLPYRDTKLGQPTIQSFEQVGTKVNVTVEDERTLVRRNNTFLSLRDVFGKDLIYTLYYWKSSSSGKKTAKTNTNEFLIDVDKGENYCFSVQAVIPSRTVNRKSTDSPVECMGQEKGEFRE

SEQ ID NO: 847 - protein, 219 aa, synthetic construct
  REGION 1..219: note = Description of Artificial Sequence: Synthetic polypeptide
SGTTNTVAAYNLTWKSTNFKTILEWEPKPVNQVYTVQISTKSGDWKSKCFYTTDTECDLTDEIVKDVKQTYLARVFSYPAGNVESTGSAGEPLYENSPEFTPYLETNIGQPVIQKYEQGGTKLKVTVKDSFTLVRKNGTFLTLRQVFGNDLGYILTYRKDSSTGRKTNTTHTNEFLIDVEKGVSYCFFAQAVIFSRKTNHKSPESITKCTEQWKSVLGE

SEQ ID NO: 848 - protein, 219 aa, synthetic construct
  REGION 1..219: note = Description of Artificial Sequence: Synthetic polypeptide
SGTTNTVAAYNLTWKSTNFKTILEWEPKPVNQVYTVQISTKSGDWKSKCFYTTDTECDLTDEIVKDVKQTYLARVFSYPAGNVESTGSAGEPLYENSPEFTPYLETNIGQPVIQKYEQGGTKLKVTVKDSFTLVRKNGTFLTLRQVFGNDLGYILTYRKSSSSGKKTAKTNTNEFLIDVDKGENYCFSVQAVIPSRTVNRKSTDSPVECMGQEKGEFRE

SEQ ID NO: 849 - protein, 219 aa, synthetic construct
  REGION 1..219: note = Description of Artificial Sequence: Synthetic polypeptide
SGTTNTVAAYNLTWKSTNFKTILEWEPKPVNQVYTVQISTKSGDWKSKCFYTTDTECDLTDEIVKDVKQTYLARVFSYPAGNVESTGSAGEPLYENSPEFTPYLETNIGQPVIQKYEQGGTKLKVTVKDSFTLVRRNNTFLSLRDVFGKDLIYTLYYWKSSSSGKKTAKTNTNEFLIDVDKGENYCFSVQAVIPSRTVNRKSTDSPVECMGQEKGEFRE

SEQ ID NO: 850 - protein, 219 aa, synthetic construct
  REGION 1..219: note = Description of Artificial Sequence: Synthetic polypeptide
SGTTNTVAAYNLTWKSTNFKTILEWEPKPVNQVYTVQISTKSGDWKSKCFYTTDTECDLTDEIVKDVKQTYLARVFSYPAGNVESTGSAGEPLYENSPEFTPYLETNLGQPTIQSFEQVGTKVNVTVEDERTLVRKNGTFLTLRQVFGNDLGYILTYRKSSSSGKKTAKTNTNEFLIDVDKGENYCFSVQAVIPSRTVNRKSTDSPVECMGQEKGEFRE

SEQ ID NO: 851 - protein, 219 aa, synthetic construct
  REGION 1..219: note = Description of Artificial Sequence: Synthetic polypeptide
SGTTNTVAAYNLTWKSTNFKTILEWEPKPVNQVYTVQISTKSGDWKSKCFYTTDTECDLTDEIVKDVKQTYLARVFSYPAGNVESTGSAGEPLYENSPEFTPYLETNLGQPTIQSFEQVGTKVNVTVEDERTLVRKNGTFLTLRQVFGKDLIYTLYYWKSSSSGKKTAKTNTNEFLIDVDKGENYCFSVQAVIPSRTVNRKSTDSPVECMGQEKGEFRE

SEQ ID NO: 852 - protein, 219 aa, synthetic construct
  REGION 1..219: note = Description of Artificial Sequence: Synthetic polypeptide
SGTTNTVAAYNLTWKSTNFKTILEWEPKPVNQVYTVQISTKSGDWKSKCFYTTDTECDLTDEIVKDVKQTYLARVFSYPAGNVESTGSAGEPLYENSPEFTPYLETNLGQPTIQSFEQVGTKVNVTVEDERTLVRKNGTFLSLRDVFGKDLIYTLYYWKSSSSGKKTAKTNTNEFLIDVDKGENYCFSVQAVIPSRTVNRKSTDSPVECMGQEKGEFRE

SEQ ID NO: 853 - protein, 219 aa, synthetic construct
  REGION 1..219: note = Description of Artificial Sequence: Synthetic polypeptide
SGTTNTVAAYNLTWKSTNFKTILEWEPKPVNQVYTVQISTKSGDWKSKCFYTTDTECDLTDEIVKDVKQTYLARVFSYPAGNVESTGSAGEPLYENSPEFTPYLETNLGQPTIQSFEQVGTKVNVTVEDERTLVRRNNTFLTLRQVFGKDLIYTLYYWKSSSSGKKTAKTNTNEFLIDVDKGENYCFSVQAVIPSRTVNRKSTDSPVECMGQEKGEFRE

SEQ ID NO: 854 - protein, 219 aa, synthetic construct
  REGION 1..219: note = Description of Artificial Sequence: Synthetic polypeptide
SGTTNTVAAYNLTWKSTNFKTILEWEPKPVNQVYTVQISTKSGDWKSKCFYTTDTECDLTDEIVKDVKQTYLARVFSYPAGNVESTGSAGEPLYENSPEFTPYLETNLGQPTIQSFEQVGTKVNVTVEDERTLVRRNNTFLSLRDVFGNDLGYILTYRKSSSSGKKTAKTNTNEFLIDVDKGENYCFSVQAVIPSRTVNRKSTDSPVECMGQEKGEFRE

SEQ ID NO: 855 - protein, 219 aa, synthetic construct
  REGION 1..219: note = Description of Artificial Sequence: Synthetic polypeptide
SGTTNTVAAYNLTWKSTNFKTILEWEPKPVNQVYTVQISTKSGDWKSKCFYTTDTECDLTDEIVKDVKQTYLARVFSYPAGNVESTGSAGEPLYENSPEFTPYLETNLGQPTIQSFEQVGTKVNVTVEDERTLVRRNNTFLSLRDVFGNDLIYTLYYWKSSSSGKKTAKTNTNEFLIDVDKGENYCFSVQAVIPSRTVNRKSTDSPVECMGQEKGEFRE

SEQ ID NO: 856 - protein, 219 aa, synthetic construct
  REGION 1..219: note = Description of Artificial Sequence: Synthetic polypeptide
SGTTNTVAAYNLTWKSTNFKTILEWEPKPVNQVYTVQISTKSGDWKSKCFYTTDTECDLTDEIVKDVKQTYLARVFSYPAGNVESTGSAGEPLYENSPEFTPYLETNLGQPTIQSFEQVGTKVNVTVEDERTLVRRNNTFLSLRDVFGKDLGYILTYRKSSSSGKKTAKTNTNEFLIDVDKGENYCFSVQAVIPSRTVNRKSTDSPVECMGQEKGEFRE

SEQ ID NO: 857 - protein, 219 aa, synthetic construct
  REGION 1..219: note = Description of Artificial Sequence: Synthetic polypeptide
SGTTNTVAAYNLTWKSTNFKTILEWEPKPVNQVYTVQISTKSGDWKSKCFYTTDTECDLTDEIVKDVKQTYLARVFSYPAGNVESTGSAGEPLYENSPEFTPYLETNLGQPTIQSFEQVGTKVNVTVEDERTLVRRNNTFLSLRDVFGKDLIYTLYYWKDSSTGRKTNTTHTNEFLIDVEKGVSYCFFAQAVIFSRKTNHKSPESITKCTEQWKSVLGE

SEQ ID NO: 858 - protein, 219 aa, synthetic construct
  REGION 1..219: note = Description of Artificial Sequence: Synthetic polypeptide
SGTTNTVAAYNLTWKSTNFKTILEWEPKPVNQVYTVQISTKSGDWKSKCFYTTDTECDLTDEIVKDVKQTYLARVFSYPAGNVESTGSAGEPLYENSPEFTPYLETNLGQPTIQSFEQVGTKVNVTVEDERTLVRRNNTFLSLRDVFGKDLIYTLYYWKDSSTGRKTNTTHTNEFLIDVEKGVSYCFFAQAVIPSRTVNRKSTDSPVECMGQEKGEFRE

SEQ ID NO: 859 - protein, 219 aa, synthetic construct
  REGION 1..219: note = Description of Artificial Sequence: Synthetic polypeptide
SGTTNTVAAYNLTWKSTNFKTILEWEPKPVNQVYTVQISTKSGDWKSKCFYTTDTECDLTDEIVKDVKQTYLARVFSYPAGNVESTGSAGEPLYENSPEFTPYLETNLGQPTIQSFEQVGTKVNVTVEDERTLVRRNNTFLSLRDVFGKDLIYTLYYWKDSSTGRKTNTTHTNEFLIDVDKGENYCFSVQAVIPSRTVNRKSTDSPVECMGQEKGEFRE

SEQ ID NO: 860 - protein, 219 aa, synthetic construct
  REGION 1..219: note = Description of Artificial Sequence: Synthetic polypeptide
SGTTNTVAAYNLTWKSTNFKTILEWEPKPVNQVYTVQISTKSGDWKSKCFYTTDTECDLTDEIVKDVKQTYLARVFSYPAGNVESTGSAGEPLYENSPEFTPYLETNLGQPTIQSFEQVGTKVNVTVEDERTLVRRNNTFLSLRDVFGKDLIYTLYYWKDSSTGRKTAKTNTNEFLIDVDKGENYCFSVQAVIPSRTVNRKSTDSPVECMGQEKGEFRE

SEQ ID NO: 861 - protein, 219 aa, synthetic construct
  REGION 1..219: note = Description of Artificial Sequence: Synthetic polypeptide
SGTTNTVAAYNLTWKSTNFKTILEWEPKPVNQVYTVQISTKSGDWKSKCFYTTDTECDLTDEIVKDVKQTYLARVFSYPAGNVESTGSAGEPLYENSPEFTPYLETNLGQPTIQSFEQVGTKVNVTVEDERTLVRRNNTFLSLRDVFGKDLIYTLYYWKSSSSGKKTNTTHTNEFLIDVDKGENYCFSVQAVIPSRTVNRKSTDSPVECMGQEKGEFRE

SEQ ID NO: 862 - protein, 219 aa, synthetic construct
  REGION 1..219: note = Description of Artificial Sequence: Synthetic polypeptide
SGTTNTVAAYNLTWKSTNFKTILEWEPKPVNQVYTVQISTKSGDWKSKCFYTTDTECDLTDEIVKDVKQTYLARVFSYPAGNVESTGSAGEPLYENSPEFTPYLETNLGQPTIQSFEQVGTKVNVTVEDERTLVRRNNTFLSLRDVFGKDLIYTLYYWKSSSSGKKTAKTNTNEFLIDVEKGVSYCFFAQAVIPSRTVNRKSTDSPVECMGQEKGEFRE

SEQ ID NO: 863 - protein, 219 aa, synthetic construct
  REGION 1..219: note = Description of Artificial Sequence: Synthetic polypeptide
SGTTNTVAAYNLTWKSTNFKTILEWEPKPVNQVYTVQISTKSGDWKSKCFYTTDTECDLTDEIVKDVKQTYLARVFSYPAGNVESTGSAGEPLYENSPEFTPYLETNLGQPTIQSFEQVGTKVNVTVEDERTLVRRNNTFLSLRDVFGKDLIYTLYYWKSSSSGKKTAKTNTNEFLIDVDKGENYCFSVQAVIFSRKTNHKSPESITKCTEQWKSVLGE

SEQ ID NO: 864 - protein, 224 aa, synthetic construct
  REGION 1..224: note = Description of Artificial Sequence: Synthetic polypeptide
AGTPPGKAFNLTWISTDFKTILEWQPKPTNYTYTVQISDRSRNWKYKCTGTTDTECDLTDEIVKDVNWTYEARVLSVPWRNSTHGKETLFGTHGEEPPFTNARKFLPYRDTKIGQPVIQKYEQGGTKLKVTVKDSFTLVRRNNTFLSLRDVFGKDLIYTLYYWKSSSSGKKTAKTNTNEFLIDVDKGENYCFSVQAVIFSRKTNHKSPESITKCTEQWKSVLGE

SEQ ID NO: 865 - protein, 219 aa, synthetic construct
  REGION 1..219: note = Description of Artificial Sequence: Synthetic polypeptide
SGTTNTVAAYNLTWKSTNFKTILEWEPKPVNQVYTVQISTKSGDWKSKCFYTTDTECDLTDEIVKDVNQTYLARVFSYPAGNVESTGSAGEPLYENSPEFTPYLETNLGQPTIQSFEQVGTKVNVTVEDERTLVRRNNTFLSLRDVFGKDLIYTLYYWKSSSSGKKTAKTNTNEFLIDVDKGENYCFSVQAVIPSRTVNRKSTDSPVECMGQEKGEFRE

SEQ ID NO: 866 - protein, 219 aa, synthetic construct; identical to SEQ ID NO: 855
  REGION 1..219: note = Description of Artificial Sequence: Synthetic polypeptide

SEQ ID NO: 867 - protein, 219 aa, synthetic construct
  REGION 1..219: note = Description of Artificial Sequence: Synthetic polypeptide
SGTTNTVAAYNLTWKSTNFKTILEWEPKPVNQVYTVQISTKSGDWKSKCFYTTDTECDLTDEIVKDVKQTYLARVFSYPAGNVESTGSAGEPLYENSPEFTPYLETNLGQPTIQSFEQVGTKVNVTVEDERTLVRRNNTFLSLRDVFGKDLIYTLYYWKSSSSGKKTAKTHTNEFLIDVDKGENYCFSVQAVIPSRKVNRKSTDSPVECMGQEKGEFRE

SEQ ID NO: 868 - protein, 123 aa, synthetic construct
  REGION 1..123: note = Description of Artificial Sequence: Synthetic polypeptide
  MOD_RES 31: note = Val or Ala
  MOD_RES 55: note = Asn or Ser
QVQLVQSGAEVKKPGASVKVSCKASGYTFDXYGISWVRQAPGQGLEWMGWIAPYXGNTNYAQKLQGRVTMTTDTSTSTAYMELRSLRSDDTAVYYCARDAGTYSPFGYGMDVWGQGTTVTVSS

SEQ ID NO: 869 - protein, 108 aa, synthetic construct
  REGION 1..108: note = Description of Artificial Sequence: Synthetic polypeptide
  MOD_RES 24: note = Arg or Gln
  MOD_RES 27: note = Gln or Glu
  MOD_RES 30: note = Ser or Asn
  MOD_RES 31: note = Ser or Asn
  MOD_RES 52: note = Ser or Tyr
  MOD_RES 53: note = Ser or Asn
  MOD_RES 56: note = Ser or Tyr
  MOD_RES 90: note = Gln or Leu
  MOD_RES 93: note = Ser or Lys
DIQMTQSPSTLSASVGDRVTITCXASXSIXXWLAWYQQKPGKAPKLLIYKAXXLEXGVPSRFSGSGSGTEFTLTISSLQPDDFATYYCQXFQXLPPFTFGGGTKVEIK

SEQ ID NO: 870 - protein, 123 aa, synthetic construct
  REGION 1..123: note = Description of Artificial Sequence: Synthetic polypeptide
  MOD_RES 55: note = Asn or Ser
QVQLVQSGAEVKKPGASVKVSCKASGYTFRSYGISWVRQAPGQGLEWMGWVAPYXGNTNYAQKLQGRVTMTTDTSTSTAYMELRSLRSDDTAVYYCARDAGTYSPYGYGMDVWGQGTTVTVSS

SEQ ID NO: 871 - protein, 108 aa, synthetic construct
  REGION 1..108: note = Description of Artificial Sequence: Synthetic polypeptide
  MOD_RES 24: note = Arg or Gln
  MOD_RES 27: note = Gln or His
  MOD_RES 30: note = Ser or Asp
  MOD_RES 50: note = Lys or Ser
  MOD_RES 53: note = Ser or Tyr
  MOD_RES 90: note = Gln, Leu, or Arg
DIQMTQSPSTLSASVGDRVTITCXASXSIXSWLAWYQQKPGKAPKLLIYXASXLESGVPSRFSGSGSGTEFTLTISSLQPDDFATYYCQXFQSLPPFTFGGGTKVEIK

SEQ ID NO: 872 - protein, 10 aa, synthetic construct
  REGION 1..10: note = Description of Artificial Sequence: Synthetic peptide
  MOD_RES 6: note = Val or Ala
GYTFDXYGIS

SEQ ID NO: 873 - protein, 17 aa, synthetic construct
  REGION 1..17: note = Description of Artificial Sequence: Synthetic peptide
  MOD_RES 6: note = Asn or Ser
WIAPYXGNTNYAQKLQG

SEQ ID NO: 874 - protein, 14 aa, synthetic construct
  REGION 1..14: note = Description of Artificial Sequence: Synthetic peptide
DAGTYSPFGYGMDV

SEQ ID NO: 875 - protein, 11 aa, synthetic construct
  REGION 1..11: note = Description of Artificial Sequence: Synthetic peptide
  MOD_RES 1: note = Arg or Gln
  MOD_RES 4: note = Gln or Glu
  MOD_RES 7: note = Ser or Asn
  MOD_RES 8: note = Ser or Asn
XASXSIXXWLA

SEQ ID NO: 876 - protein, 7 aa, synthetic construct
  REGION 1..7: note = Description of Artificial Sequence: Synthetic peptide
  MOD_RES 3: note = Ser or Tyr
  MOD_RES 4: note = Ser or Asn
  MOD_RES 7: note = Ser or Tyr
KAXXLEX

SEQ ID NO: 877 - protein, 10 aa, synthetic construct
  REGION 1..10: note = Description of Artificial Sequence: Synthetic peptide
  MOD_RES 2: note = Gln or Leu
  MOD_RES 5: note = Ser or Lys
QXFQXLPPFT

SEQ ID NO: 878 - protein, 10 aa, synthetic construct
  REGION 1..10: note = Description of Artificial Sequence: Synthetic peptide
GYTFRSYGIS

SEQ ID NO: 879 - protein, 17 aa, synthetic construct
  REGION 1..17: note = Description of Artificial Sequence: Synthetic peptide
  MOD_RES 6: note = Asn or Ser
WVAPYXGNTNYAQKLQG

SEQ ID NO: 880 - protein, 14 aa, synthetic construct
  REGION 1..14: note = Description of Artificial Sequence: Synthetic peptide
DAGTYSPYGYGMDV

SEQ ID NO: 881 - protein, 11 aa, synthetic construct
  REGION 1..11: note = Description of Artificial Sequence: Synthetic peptide
  MOD_RES 1: note = Arg or Gln
  MOD_RES 4: note = Gln or His
  MOD_RES 7: note = Ser or Asp
XASXSIXSWLA

SEQ ID NO: 882 - protein, 7 aa, synthetic construct
  REGION 1..7: note = Description of Artificial Sequence: Synthetic peptide
  MOD_RES 1: note = Lys or Ser
  MOD_RES 4: note = Ser or Tyr
XASXLES

SEQ ID NO: 883 - protein, 10 aa, synthetic construct
  REGION 1..10: note = Description of Artificial Sequence: Synthetic peptide
  MOD_RES 2: note = Gln, Leu, or Arg
QXFQSLPPFT

SEQ ID NO: 884 - protein, 10 aa, synthetic construct
  REGION 1..10: note = Description of Artificial Sequence: Synthetic peptide
GYTFDAYGIS

SEQ ID NO: 885 - protein, 17 aa, synthetic construct
  REGION 1..17: note = Description of Artificial Sequence: Synthetic peptide
WIAPYSGNTNYAQKLQG

SEQ ID NO: 886 - protein, 14 aa, synthetic construct
  REGION 1..14: note = Description of Artificial Sequence: Synthetic peptide
DAGTYSPFGYGMDV

SEQ ID NO: 887 - protein, 11 aa, synthetic construct
  REGION 1..11: note = Description of Artificial Sequence: Synthetic peptide
RASESISNWLA

SEQ ID NO: 888 - protein, 7 aa, synthetic construct
  REGION 1..7: note = Description of Artificial Sequence: Synthetic peptide
KAYSLEY

SEQ ID NO: 889 - protein, 10 aa, synthetic construct
  REGION 1..10: note = Description of Artificial Sequence: Synthetic peptide
QQFQKLPPFT

SEQ ID NO: 890 - protein, 5 aa, synthetic construct
  REGION 1..5: note = Description of Artificial Sequence: Synthetic peptide
AYGIS

SEQ ID NO: 891 - protein, 17 aa, synthetic construct
  REGION 1..17: note = Description of Artificial Sequence: Synthetic peptide
WIAPYSGNTNYAQKLQG

SEQ ID NO: 892 - protein, 14 aa, synthetic construct
  REGION 1..14: note = Description of Artificial Sequence: Synthetic peptide
DAGTYSPFGYGMDV

SEQ ID NO: 893 - protein, 11 aa, synthetic construct
  REGION 1..11: note = Description of Artificial Sequence: Synthetic peptide
RASESISNWLA

SEQ ID NO: 894 - protein, 7 aa, synthetic construct
  REGION 1..7: note = Description of Artificial Sequence: Synthetic peptide
KAYSLEY

SEQ ID NO: 895 - protein, 10 aa, synthetic construct
  REGION 1..10: note = Description of Artificial Sequence: Synthetic peptide
QQFQKLPPFT

SEQ ID NO: 896 - protein, 7 aa, synthetic construct
  REGION 1..7: note = Description of Artificial Sequence: Synthetic peptide
GYTFDAY

SEQ ID NO: 897 - protein, 4 aa, synthetic construct
  REGION 1..4: note = Description of Artificial Sequence: Synthetic peptide
PYSG

SEQ ID NO: 898 - protein, 12 aa, synthetic construct
  REGION 1..12: note = Description of Artificial Sequence: Synthetic peptide
AGTYSPFGYGMD

SEQ ID NO: 899 - protein, 7 aa, synthetic construct
  REGION 1..7: note = Description of Artificial Sequence: Synthetic peptide
SESISNW

SEQ ID NO: 900 - skipped

SEQ ID NO: 901 - protein, 7 aa, synthetic construct
  REGION 1..7: note = Description of Artificial Sequence: Synthetic peptide
FQKLPPF

SEQ ID NO: 902 - protein, 10 aa, synthetic construct
  REGION 1..10: note = Description of Artificial Sequence: Synthetic peptide
GYTFDAYGIS

SEQ ID NO: 903 - protein, 10 aa, synthetic construct
  REGION 1..10: note = Description of Artificial Sequence: Synthetic peptide
WIAPYSGNTN

SEQ ID NO: 904 - protein, 14 aa, synthetic construct
  REGION 1..14: note = Description of Artificial Sequence: Synthetic peptide
DAGTYSPFGYGMDV

SEQ ID NO: 905 - protein, 11 aa, synthetic construct
  REGION 1..11: note = Description of Artificial Sequence: Synthetic peptide
RASESISNWLA

SEQ ID NO: 906 - protein, 7 aa, synthetic construct
  REGION 1..7: note = Description of Artificial Sequence: Synthetic peptide
KAYSLEY

SEQ ID NO: 907 - protein, 10 aa, synthetic construct
  REGION 1..10: note = Description of Artificial Sequence: Synthetic peptide
QQFQKLPPFT

SEQ ID NO: 908 - protein, 6 aa, synthetic construct
  REGION 1..6: note = Description of Artificial Sequence: Synthetic peptide
DAYGIS

SEQ ID NO: 909 - protein, 13 aa, synthetic construct
  REGION 1..13: note = Description of Artificial Sequence: Synthetic peptide
WMGWIAPYSGNTN

SEQ ID NO: 910 - protein, 15 aa, synthetic construct
  REGION 1..15: note = Description of Artificial Sequence: Synthetic peptide
ARDAGTYSPFGYGMD

SEQ ID NO: 911 - protein, 7 aa, synthetic construct
  REGION 1..7: note = Description of Artificial Sequence: Synthetic peptide
SNWLAWY

SEQ ID NO: 912 - protein, 10 aa, synthetic construct
  REGION 1..10: note = Description of Artificial Sequence: Synthetic peptide
LLIYKAYSLE

SEQ ID NO: 913 - protein, 9 aa, synthetic construct
  REGION 1..9: note = Description of Artificial Sequence: Synthetic peptide
QQFQKLPPF

SEQ ID NO: 914 - protein, 8 aa, synthetic construct
  REGION 1..8: note = Description of Artificial Sequence: Synthetic peptide
GYTFDAYG

SEQ ID NO: 915 - protein, 8 aa, synthetic construct
  REGION 1..8: note = Description of Artificial Sequence: Synthetic peptide
IAPYSGNT

SEQ ID NO: 916 - protein, 16 aa, synthetic construct
  REGION 1..16: note = Description of Artificial Sequence: Synthetic peptide
ARDAGTYSPFGTGMDV

SEQ ID NO: 917 - protein, 6 aa, synthetic construct
  REGION 1..6: note = Description of Artificial Sequence: Synthetic peptide
ESISNW

SEQ ID NO: 918 - skipped

SEQ ID NO: 919 - protein, 10 aa, synthetic construct
  REGION 1..10: note = Description of Artificial Sequence: Synthetic peptide
QQFQKLPPFT

SEQ ID NO: 920 - protein, 4 aa, Homo sapiens
ELLG

SEQ ID NO: 921 - protein, 4 aa, Homo sapiens
EFLG

SEQ ID NO: 922 - protein, 6 aa, synthetic construct
  REGION 1..6: note = Description of Artificial Sequence: Synthetic 6xHis tag
HHHHHH